European Patent Specification EP 3 813 522 B1, published May 7, 2025. Title: Models Of Tauopathy. Applicant: Regeneron Pharmaceuticals, Inc. The sequence listing filed with the application follows.

SEQUENCE LISTING (324 sequences)

SEQ ID NO: 1 - DNA, 20 bp, Homo sapiens
ttgcaggcctatgttgtcct

SEQ ID NO: 2 - DNA, 20 bp, Homo sapiens
gcttcggatgccttcgagag

SEQ ID NO: 3 - DNA, 20 bp, Homo sapiens
tttcctccagcttcttgccc

SEQ ID NO: 4 - DNA, 20 bp, Homo sapiens
cgccaacgccaagcagtccc

SEQ ID NO: 5 - DNA, 20 bp, Homo sapiens
gagctctagacaccaacgtg

SEQ ID NO: 6 - DNA, 20 bp, Homo sapiens
caagcagctgtccgagtccc

SEQ ID NO: 7 - DNA, 20 bp, Artificial Sequence
  Synthetic
cttcgacgccatcgtgctca

SEQ ID NO: 8 - DNA, 20 bp, Artificial Sequence
  Synthetic
cgcctctcacgtgtaggctt

SEQ ID NO: 9 - DNA, 20 bp, Homo sapiens
tttaaggaacccagtgacaa

SEQ ID NO: 10 - DNA, 20 bp, Homo sapiens
ggccttgaacacagttccgt

SEQ ID NO: 11 - DNA, 20 bp, Homo sapiens
tagagttgtcatctttcaac

SEQ ID NO: 12 - DNA, 20 bp, Homo sapiens
aaggagccgcccctgtacta

SEQ ID NO: 13 - DNA, 20 bp, Homo sapiens
tccggccaggatcaactcgt

SEQ ID NO: 14 - DNA, 20 bp, Homo sapiens
tacttacggctatatattct

SEQ ID NO: 15 - DNA, 20 bp, Homo sapiens
aagaacgctttctgttcaag

SEQ ID NO: 16 - DNA, 20 bp, Homo sapiens
gtgaaatacggagtgaatcc

SEQ ID NO: 17 - DNA, 20 bp, Artificial Sequence
  Synthetic
atagccgccgctcattactt

SEQ ID NO: 18 - DNA, 20 bp, Mus musculus
atgaagacctcttccgagaa

SEQ ID NO: 19 - DNA, 20 bp, Mus musculus
atcccggccaggctccccac

SEQ ID NO: 20 - DNA, 20 bp, Mus musculus
ttggtgacgtcctgagcaag

SEQ ID NO: 21 - DNA, 20 bp, Mus musculus
ccgagcactcgatcgcctac

SEQ ID NO: 22 - DNA, 20 bp, Mus musculus
acatcgaacctcttgaacgt

SEQ ID NO: 23 - DNA, 20 bp, Mus musculus
gggatatctcctcggggagc

SEQ ID NO: 24 - DNA, 20 bp, Mus musculus
gatacaggtcaacaacgtag

SEQ ID NO: 25 - DNA, 20 bp, Mus musculus
ttcgacagctttccgcagct

SEQ ID NO: 26 - DNA, 20 bp, Mus musculus
ccagaaccaattagatatcg

SEQ ID NO: 27 - RNA, 20 nt, Artificial Sequence
  Synthetic
uugcaggccuauguuguccu

SEQ ID NO: 28 - RNA, 20 nt, Artificial Sequence
  Synthetic
gcuucggaugccuucgagag

SEQ ID NO: 29 - RNA, 20 nt, Artificial Sequence
  Synthetic
uuuccuccagcuucuugccc

SEQ ID NO: 30 - RNA, 20 nt, Artificial Sequence
  Synthetic
cgccaacgccaagcaguccc

SEQ ID NO: 31 - RNA, 20 nt, Artificial Sequence
  Synthetic
gagcucuagacaccaacgug

SEQ ID NO: 32 - RNA, 20 nt, Artificial Sequence
  Synthetic
caagcagcuguccgaguccc

SEQ ID NO: 33 - RNA, 20 nt, Artificial Sequence
  Synthetic
cuucgacgccaucgugcuca

SEQ ID NO: 34 - RNA, 20 nt, Artificial Sequence
  Synthetic
cgccucucacguguaggcuu

SEQ ID NO: 35 - RNA, 20 nt, Artificial Sequence
  Synthetic
uuuaaggaacccagugacaa

SEQ ID NO: 36 - RNA, 20 nt, Artificial Sequence
  Synthetic
ggccuugaacacaguuccgu

SEQ ID NO: 37 - RNA, 20 nt, Artificial Sequence
  Synthetic
uagaguugucaucuuucaac

SEQ ID NO: 38 - RNA, 20 nt, Artificial Sequence
  Synthetic
aaggagccgccccuguacua

SEQ ID NO: 39 - RNA, 20 nt, Artificial Sequence
  Synthetic
uccggccaggaucaacucgu

SEQ ID NO: 40 - RNA, 20 nt, Artificial Sequence
  Synthetic
uacuuacggcuauauauucu

SEQ ID NO: 41 - RNA, 20 nt, Artificial Sequence
  Synthetic
aagaacgcuuucuguucaag

SEQ ID NO: 42 - RNA, 20 nt, Artificial Sequence
  Synthetic
gugaaauacggagugaaucc

SEQ ID NO: 43 - RNA, 20 nt, Artificial Sequence
  Synthetic
auagccgccgcucauuacuu

SEQ ID NO: 44 - RNA, 20 nt, Artificial Sequence
  Synthetic
augaagaccucuuccgagaa

SEQ ID NO: 45 - RNA, 20 nt, Artificial Sequence
  Synthetic
aucccggccaggcuccccac

SEQ ID NO: 46 - RNA, 20 nt, Artificial Sequence
  Synthetic
uuggugacguccugagcaag

SEQ ID NO: 47 - RNA, 20 nt, Artificial Sequence
  Synthetic
ccgagcacucgaucgccuac

SEQ ID NO: 48 - RNA, 20 nt, Artificial Sequence
  Synthetic
acaucgaaccucuugaacgu

SEQ ID NO: 49 - RNA, 20 nt, Artificial Sequence
  Synthetic
gggauaucuccucggggagc

SEQ ID NO: 50 - RNA, 20 nt, Artificial Sequence
  Synthetic
gauacaggucaacaacguag

SEQ ID NO: 51 - RNA, 20 nt, Artificial Sequence
  Synthetic
uucgacagcuuuccgcagcu

SEQ ID NO: 52 - RNA, 20 nt, Artificial Sequence
  Synthetic
ccagaaccaauuagauaucg

SEQ ID NO: 53 - DNA, 21 bp, Artificial Sequence
  Synthetic
agaatctgaagcatcaaccgg

SEQ ID NO: 54 - DNA, 22 bp, Artificial Sequence
  Synthetic
ggtttgtaaacgatctgcactg

SEQ ID NO: 55 - DNA, 24 bp, Artificial Sequence
  Synthetic
aatatcaagcacgtccctggaggc

SEQ ID NO: 56 - DNA, 21 bp, Artificial Sequence
  Synthetic
ccgaaaatctcaagcatcagc

SEQ ID NO: 57 - DNA, 20 bp, Artificial Sequence
  Synthetic
acacaatctgtacgcttccg

SEQ ID NO: 58 - DNA, 24 bp, Artificial Sequence
  Synthetic
tgcacgttagacaggtccagcttc

SEQ ID NO: 59 - DNA, 24 bp, Artificial Sequence
  Synthetic
ggcggtaaggtccaaattataaac

SEQ ID NO: 60 - DNA, 22 bp, Artificial Sequence
  Synthetic
ggtttgtaaacgatctgaacgg

SEQ ID NO: 61 - DNA, 24 bp, Artificial Sequence
  Synthetic
aatgtccaaagcaagtgtggcagc

SEQ ID NO: 62 - DNA, 22 bp, Artificial Sequence
  Synthetic
ggtagtacagagaacctgaagc

SEQ ID NO: 63 - DNA, 20 bp, Artificial Sequence
  Synthetic
ctttgctcccacatttgctc

SEQ ID NO: 64 - DNA, 24 bp, Artificial Sequence
  Synthetic
cggtggtggtaaggtccagatcat

SEQ ID NO: 65 - RNA, 16 nt, Artificial Sequence
  Synthetic
guuuuagagcuaugcu

SEQ ID NO: 66 - RNA, 67 nt, Artificial Sequence
  Synthetic
agcauagcaaguuaaaauaaggcuaguccguuaucaacuugaaaaaguggcaccgagucggugcuuu

SEQ ID NO: 67 - RNA, 77 nt, Artificial Sequence
  Synthetic
guuuuagagcuagaaauagcaaguuaaaauaaggcuaguccguuaucaacuugaaaaaguggcaccgagucggugcu

SEQ ID NO: 68 - RNA, 82 nt, Artificial Sequence
  Synthetic
guuggaaccauucaaaacagcauagcaaguuaaaauaaggcuaguccguuaucaacuugaaaaaguggcaccgagucggugc

SEQ ID NO: 69 - RNA, 76 nt, Artificial Sequence
  Synthetic
guuuuagagcuagaaauagcaaguuaaaauaaggcuaguccguuaucaacuugaaaaaguggcaccgagucggugc

SEQ ID NO: 70 - RNA, 86 nt, Artificial Sequence
  Synthetic
guuuaagagcuaugcuggaaacagcauagcaaguuuaaauaaggcuaguccguuaucaacuugaaaaaguggcaccgagucggugc

SEQ ID NO: 71 - DNA, 23 bp, Artificial Sequence
  Synthetic
  misc_feature (2)..(21): n is a, c, g, or t
gnnnnnnnnnnnnnnnnnnnngg

SEQ ID NO: 72 - DNA, 23 bp, Artificial Sequence
  Synthetic
  misc_feature (1)..(21): n is a, c, g, or t
nnnnnnnnnnnnnnnnnnnnngg

SEQ ID NO: 73 - DNA, 25 bp, Artificial Sequence
  Synthetic
  misc_feature (3)..(23): n is a, c, g, or t
ggnnnnnnnnnnnnnnnnnnnnngg

SEQ ID NO: 74 - DNA, 9099 bp, Artificial Sequence
  Synthetic
  misc_feature (1)..(635): LTR
  misc_feature (636)..(653): PBS
  misc_feature (685)..(822): Packaging\signal
  misc_feature (1303)..(1536): RRE
  misc_feature (2028)..(2151): cPPT
  misc_feature (2185)..(2668): hSynapsin promoter
  misc_feature (2675)..(2686): MCS
  misc_feature (2687)..(3403): GFP
  misc_feature (3415)..(3420): MCS
  misc_feature (3421)..(4019): IRES
  misc_feature (4020)..(5054): HygR
  misc_feature (5068)..(5659): WPRE
  misc_feature (5862)..(6498): LTR
  misc_feature (6967)..(7640): pUC\origin
  misc_feature (7785)..(8781): AmpR
tggaagggctaattcactcccaaagaagacaagatatccttgatctgtggatctaccacacacaaggctacttccctgattagcagaactacacaccagggccaggggtcagatatccactgacctttggatggtgctacaagctagtaccagttgagccagataaggtagaagaggccaataaaggagagaacaccagcttgttacaccctgtgagcctgcatgggatggatgacccggagagagaagtgttagagtggaggtttgacagccgcctagcatttcatcacgtggcccgagagctgcatccggagtacttcaagaactgctgatatcgagcttgctacaagggactttccgctggggactttccagggaggcgtggcctgggcgggactggggagtggcgagccctcagatcctgcatataagcagctgctttttgcctgtactgggtctctctggttagaccagatctgagcctgggagctctctggctaactagggaacccactgcttaagcctcaataaagcttgccttgagtgcttcaagtagtgtgtgcccgtctgttgtgtgactctggtaactagagatccctcagacccttttagtcagtgtggaaaatctctagcagtggcgcccgaacagggacttgaaagcgaaagggaaaccagaggagctctctcgacgcaggactcggcttgctgaagcgcgcacggcaagaggcgaggggcggcgactggtgagtacgccaaaaattttgactagcggaggctagaaggagagagatgggtgcgagagcgtcagtattaagcgggggagaattagatcgcgatgggaaaaaattcggttaaggccagggggaaagaaaaaatataaattaaaacatatagtatgggcaagcagggagctagaacgattcgcagttaatcctggcctgttagaaacatcagaaggctgtagacaaatactgggacagctacaaccatcccttcagacaggatcagaagaacttagatcattatataatacagtagcaaccctctattgtgtgcatcaaaggatagagataaaagacaccaaggaagctttagacaagatagaggaagagcaaaacaaaagtaagaccaccgcacagcaagcggccggccgctgatcttcagacctggaggaggagatatgagggacaattggagaagtgaattatataaatataaagtagtaaaaattgaaccattaggagtagcacccaccaaggcaaagagaagagtggtgcagagagaaaaaagagcagtgggaataggagctttgttccttgggttcttgggagcagcaggaagcactatgggcgcagcgtcaatgacgctgacggtacaggccagacaattattgtctggtatagtgcagcagcagaacaatttgctgagggctattgaggcgcaacagcatctgttgcaactcacagtctggggcatcaagcagctccaggcaagaatcctggctgtggaaagatacctaaaggatcaacagctcctggggatttggggttgctctggaaaactcatttgcaccactgctgtgccttggaatgctagttggagtaataaatctctggaacagatttggaatcacacgacctggatggagtgggacagagaaattaacaattacacaagcttaatacactccttaattgaagaatcgcaaaaccagcaagaaaagaatgaacaagaattattggaattagataaatgggcaagtttgtggaattggtttaacataacaaattggctgtggtatataaaattattcataatgatagtaggaggcttggtaggtttaagaatagtttttgctgtactttctatagtgaatagagttaggcagggatattcaccattatcgtttcagacccacctcccaaccccgaggggacccgacaggcccgaaggaatagaagaagaaggtggagagagagacagagacagatccattcgattagtgaacggatctcgacggtatcgcctttaaaagaaaaggggggattggggggtacagtgcaggggaaagaatagtagacataatagcaacagacatacaaactaaagaattacaaaaacaaattacaaaaattcaaaattttcgggtttattacagggacagcagagatccagtttatcgatctgcagagggccctgcgtatgagtgcaagtgggttttaggaccaggatgaggcggggtgggggtgcctacctgacgaccgaccccgacccactggacaagcacccaacccccattccccaaattgcgcatcccctatcagagagggggaggggaaacaggatgcggcgaggcgcgtgcgcactgccagcttcagcaccgcggacagtgccttcgcccccgcctggcggcgcgcgccaccgccgcctcagcactgaaggcgcgctgacgtcactcgccggtcccccgcaaactccccttcccggccaccttggtcgcgtccgcgccgccgccggcccagccggaccgcaccacgcgaggcgcgagataggggggcacgggcgcgaccatctgcgctgcggcgccggcgactcagcgctgcctcagtctgcggtgggcagcggaggagtcgtgtcgtgcctgagagcgcagggatctatttccggtgaattcctcgagactagtatggtgagcaagggcgaggagctgttcaccggggtggtgcccatcctggtcgagctggacggcgacgtaaacggccacaagttcagcgtgtccggcgagggcgagggcgatgccacctacggcaagctgaccctgaagttcatctgcaccaccggcaagctgcccgtgccctggcccaccctcgtgaccaccctgacctacggcgtgcagtgcttcagccgctaccccgaccacatgaagcagcacgacttcttcaagtccgccatgcccgaaggctacgtccaggagcgcaccatcttcttcaaggacgacggcaactacaagacccgcgccgaggtgaagttcgagggcgacaccctggtgaaccgcatcgagctgaagggcatcgacttcaaggaggacggcaacatcctggggcacaagctggagtacaactacaacagccacaacgtctatatcatggccgacaagcagaagaacggcatcaaggtgaacttcaagatccgccacaacatcgaggacggcagcgtgcagctcgccgaccactaccagcagaacacccccatcggcgacggccccgtgctgctgcccgacaaccactacctgagcacccagtccgccctgagcaaagaccccaacgagaagcgcgatcacatggtcctgctggagttcgtgaccgccgccgggatcactctcggcatggacgagctgtacaagtaagcggccgcggatcccgcccctctccctcccccccccctaacgttactggccgaagccgcttggaataaggccggtgtgcgtttgtctatatgttattttccaccatattgccgtcttttggcaatgtgagggcccggaaacctggccctgtcttcttgacgagcattcctaggggtctttcccctctcgccaaaggaatgcaaggtctgttgaatgtcgtgaaggaagcagttcctctggaagcttcttgaagacaaacaacgtctgtagcgaccctttgcaggcagcggaaccccccacctggcgacaggtgcctctgcggccaaaagccacgtgtataagatacacctgcaaaggcggcacaaccccagtgccacgttgtgagttggatagttgtggaaagagtcaaatggctctcctcaagcgtattcaacaaggggctgaaggatgcccagaaggtaccccattgtatgggatctgatctggggcctcggtgcacatgctttacatgtgtttagtcgaggttaaaaaaacgtctaggccccccgaaccacggggacgtggttttcctttgaaaaacacgatgataagcttgccacaacccgtaccaaagatggatagatccggaaagcctgaactcaccgcgacgtctgtcgagaagtttctgatcgaaaagttcgacagcgtctccgacctgatgcagctctcggagggcgaagaatctcgtgctttcagcttcgatgtaggagggcgtggatatgtcctgcgggtaaatagctgcgccgatggtttctacaaagatcgttatgtttatcggcactttgcatcggccgcgctcccgattccggaagtgcttgacattggggaattcagcgagagcctgacctattgcatctcccgccgtgcacagggtgtcacgttgcaagacctgcctgaaaccgaactgcccgctgttctgcagccggtcgcggaggccatggatgcgatcgctgcggccgatcttagccagacgagcgggttcggcccattcggaccgcaaggaatcggtcaatacactacatggcgtgatttcatatgcgcgattgctgatccccatgtgtatcactggcaaactgtgatggacgacaccgtcagtgcgtccgtcgcgcaggctctcgatgagctgatgctttgggccgaggactgccccgaagtccggcacctcgtgcacgcggatttcggctccaacaatgtcctgacggacaatggccgcataacagcggtcattgactggagcgaggcgatgttcggggattcccaatacgaggtcgccaacatcttcttctggaggccgtggttggcttgtatggagcagcagacgcgctacttcgagcggaggcatccggagcttgcaggatcgccgcggctccgggcgtatatgctccgcattggtcttgaccaactctatcagagcttggttgacggcaatttcgatgatgcagcttgggcgcagggtcgatgcgacgcaatcgtccgatccggagccgggactgtcgggcgtacacaaatcgcccgcagaagcgcggccgtctggaccgatggctgtgtagaagtactcgccgatagtggaaaccgacgccccagcactcgtccgagggcaaaggaatagacgcgtctggaacaatcaacctctggattacaaaatttgtgaaagattgactggtattcttaactatgttgctccttttacgctatgtggatacgctgctttaatgcctttgtatcatgctattgcttcccgtatggctttcattttctcctccttgtataaatcctggttgctgtctctttatgaggagttgtggcccgttgtcaggcaacgtggcgtggtgtgcactgtgtttgctgacgcaacccccactggttggggcattgccaccacctgtcagctcctttccgggactttcgctttccccctccctattgccacggcggaactcatcgccgcctgccttgcccgctgctggacaggggctcggctgttgggcactgacaattccgtggtgttgtcggggaagctgacgtcctttccatggctgctcgcctgtgttgccacctggattctgcgcgggacgtccttctgctacgtcccttcggccctcaatccagcggaccttccttcccgcggcctgctgccggctctgcggcctcttccgcgtcttcgccttcgccctcagacgagtcggatctccctttgggccgcctccccgcctggaattaattctgcagtcgagacctagaaaaacatggagcaatcacaagtagcaatacagcagctaccaatgctgattgtgcctggctagaagcacaagaggaggaggaggtgggttttccagtcacacctcaggtacctttaagaccaatgacttacaaggcagctgtagatcttagccactttttaaaagaaaagaggggactggaagggctaattcactcccaacgaagacaagatatccttgatctgtggatctaccacacacaaggctacttccctgattagcagaactacacaccagggccaggggtcagatatccactgacctttggatggtgctacaagctagtaccagttgagccagataaggtagaagaggccaataaaggagagaacaccagcttgttacaccctgtgagcctgcatgggatggatgacccggagagagaagtgttagagtggaggtttgacagccgcctagcatttcatcacgtggcccgagagctgcatccggagtacttcaagaactgctgatatcgagcttgctacaagggactttccgctggggactttccagggaggcgtggcctgggcgggactggggagtggcgagccctcagatcctgcatataagcagctgctttttgcctgtactgggtctctctggttagaccagatctgagcctgggagctctctggctaactagggaacccactgcttaagcctcaataaagcttgccttgagtgcttcaagtagtgtgtgcccgtctgttgtgtgactctggtaactagagatccctcagacccttttagtcagtgtggaaaatctctagcagtagtagttcatgtcatcttattattcagtatttataacttgcaaagaaatgaatatcagagagtgagaggccttgacattgctagcgtttaccgtcgacctctagctagagcttggcgtaatcatggtcatagctgtttcctgtgtgaaattgttatccgctcacaattccacacaacatacgagccggaagcataaagtgtaaagcctggggtgcctaatgagtgagctaactcacattaattgcgttgcgctcactgcccgctttccagtcgggaaacctgtcgtgccagctgcattaatgaatcggccaacgcgcggggagaggcggtttgcgtattgggcgctcttccgcttcctcgctcactgactcgctgcgctcggtcgttcggctgcggcgagcggtatcagctcactcaaaggcggtaatacggttatccacagaatcaggggataacgcaggaaagaacatgtgagcaaaaggccagcaaaaggccaggaaccgtaaaaaggccgcgttgctggcgtttttccataggctccgcccccctgacgagcatcacaaaaatcgacgctcaagtcagaggtggcgaaacccgacaggactataaagataccaggcgtttccccctggaagctccctcgtgcgctctcctgttccgaccctgccgcttaccggatacctgtccgcctttctcccttcgggaagcgtggcgctttctcatagctcacgctgtaggtatctcagttcggtgtaggtcgttcgctccaagctgggctgtgtgcacgaaccccccgttcagcccgaccgctgcgccttatccggtaactatcgtcttgagtccaacccggtaagacacgacttatcgccactggcagcagccactggtaacaggattagcagagcgaggtatgtaggcggtgctacagagttcttgaagtggtggcctaactacggctacactagaagaacagtatttggtatctgcgctctgctgaagccagttaccttcggaaaaagagttggtagctcttgatccggcaaacaaaccaccgctggtagcggtggtttttttgtttgcaagcagcagattacgcgcagaaaaaaaggatctcaagaagatcctttgatcttttctacggggtctgacgctcagtggaacgaaaactcacgttaagggattttggtcatgagattatcaaaaaggatcttcacctagatccttttaaattaaaaatgaagttttaaatcaatctaaagtatatatgagtaaacttggtctgacagttaccaatgcttaatcagtgaggcacctatctcagcgatctgtctatttcgttcatccatagttgcctgactccccgtcgtgtagataactacgatacgggagggcttaccatctggccccagtgctgcaatgataccgcgagacccacgctcaccggctccagatttatcagcaataaaccagccagccggaagggccgagcgcagaagtggtcctgcaactttatccgcctccatccagtctattaattgttgccgggaagctagagtaagtagttcgccagttaatagtttgcgcaacgttgttgccattgctacaggcatcgtggtgtcacgctcgtcgtttggtatggcttcattcagctccggttcccaacgatcaaggcgagttacatgatcccccatgttgtgcaaaaaagcggttagctccttcggtcctccgatcgttgtcagaagtaagttggccgcagtgttatcactcatggttatggcagcactgcataattctcttactgtcatgccatccgtaagatgcttttctgtgactggtgagtactcaaccaagtcattctgagaatagtgtatgcggcgaccgagttgctcttgcccggcgtcaatacgggataataccgcgccacatagcagaactttaaaagtgctcatcattggaaaacgttcttcggggcgaaaactctcaaggatcttaccgctgttgagatccagttcgatgtaacccactcgtgcacccaactgatcttcagcatcttttactttcaccagcgtttctgggtgagcaaaaacaggaaggcaaaatgccgcaaaaaagggaataagggcgacacggaaatgttgaatactcatactcttcctttttcaatattattgaagcatttatcagggttattgtctcatgagcggatacatatttgaatgtatttagaaaaataaacaaataggggttccgcgcacatttccccgaaaagtgccacctgacgtcgacggatcgggagatcaacttgtttattgcagcttataatggttacaaataaagcaatagcatcacaaatttcacaaataaagcatttttttcactgcattctagttgtggtttgtccaaactcatcaatgtatcttatcatgtctggatcaactggataactcaagctaaccaaaatcatcccaaacttcccaccccataccctattaccactgccaattacctgtggtttcatttactctaaacctgtgattcctctgaattattttcattttaaagaaattgtatttgttaaatatgtactacaaacttagtagt

SEQ ID NO: 75 - DNA, 9636 bp, Artificial Sequence
  Synthetic
  misc_feature (1)..(635): LTR
  misc_feature (636)..(653): PBS
  misc_feature (685)..(822): Packaging\signal
  misc_feature (1303)..(1536): RRE
  misc_feature (2028)..(2151): cPPT
  misc_feature (2185)..(2668): hSynapsin promoter
  misc_feature (2681)..(3919): hTau-412 (1N4R) WT
  misc_feature (3926)..(3957): MCS
  misc_feature (3958)..(4556): IRES
  misc_feature (4557)..(5591): HygR
  misc_feature (5605)..(6196): WPRE
  misc_feature (6399)..(7035): LTR
  misc_feature (7504)..(8177): pUC\origin
  misc_feature (8322)..(9318): AmpR
tggaagggctaattcactcccaaagaagacaagatatccttgatctgtggatctaccacacacaaggctacttccctgattagcagaactacacaccagggccaggggtcagatatccactgacctttggatggtgctacaagctagtaccagttgagccagataaggtagaagaggccaataaaggagagaacaccagcttgttacaccctgtgagcctgcatgggatggatgacccggagagagaagtgttagagtggaggtttgacagccgcctagcatttcatcacgtggcccgagagctgcatccggagtacttcaagaactgctgatatcgagcttgctacaagggactttccgctggggactttccagggaggcgtggcctgggcgggactggggagtggcgagccctcagatcctgcatataagcagctgctttttgcctgtactgggtctctctggttagaccagatctgagcctgggagctctctggctaactagggaacccactgcttaagcctcaataaagcttgccttgagtgcttcaagtagtgtgtgcccgtctgttgtgtgactctggtaactagagatccctcagacccttttagtcagtgtggaaaatctctagcagtggcgcccgaacagggacttgaaagcgaaagggaaaccagaggagctctctcgacgcaggactcggcttgctgaagcgcgcacggcaagaggcgaggggcggcgactggtgagtacgccaaaaattttgactagcggaggctagaaggagagagatgggtgcgagagcgtcagtattaagcgggggagaattagatcgcgatgggaaaaaattcggttaaggccagggggaaagaaaaaatataaattaaaacatatagtatgggcaagcagggagctagaacgattcgcagttaatcctggcctgttagaaacatcagaaggctgtagacaaatactgggacagctacaaccatcccttcagacaggatcagaagaacttagatcattatataatacagtagcaaccctctattgtgtgcatcaaaggatagagataaaagacaccaaggaagctttagacaagatagaggaagagcaaaacaaaagtaagaccaccgcacagcaagcggccggccgctgatcttcagacctggaggaggagatatgagggacaattggagaagtgaattatataaatataaagtagtaaaaattgaaccattaggagtagcacccaccaaggcaaagagaagagtggtgcagagagaaaaaagagcagtgggaataggagctttgttccttgggttcttgggagcagcaggaagcactatgggcgcagcgtcaatgacgctgacggtacaggccagacaattattgtctggtatagtgcagcagcagaacaatttgctgagggctattgaggcgcaacagcatctgttgcaactcacagtctggggcatcaagcagctccaggcaagaatcctggctgtggaaagatacctaaaggatcaacagctcctggggatttggggttgctctggaaaactcatttgcaccactgctgtgccttggaatgctagttggagtaataaatctctggaacagatttggaatcacacgacctggatggagtgggacagagaaattaacaattacacaagcttaatacactccttaattgaagaatcgcaaaaccagcaagaaaagaatgaacaagaattattggaattagataaatgggcaagtttgtggaattggtttaacataacaaattggctgtggtatataaaattattcataatgatagtaggaggcttggtaggtttaagaatagtttttgctgtactttctatagtgaatagagttaggcagggatattcaccattatcgtttcagacccacctcccaaccccgaggggacccgacaggcccgaaggaatagaagaagaaggtggagagagagacagagacagatccattcgattagtgaacggatctcgacggtatcgcctttaaaagaaaaggggggattggggggtacagtgcaggggaaagaatagtagacataatagcaacagacatacaaactaaagaattacaaaaacaaattacaaaaattcaaaattttcgggtttattacagggacagcagagatccagtttatcgatctgcagagggccctgcgtatgagtgcaagtgggttttaggaccaggatgaggcggggtgggggtgcctacctgacgaccgaccccgacccactggacaagcacccaacccccattccccaaattgcgcatcccctatcagagagggggaggggaaacaggatgcggcgaggcgcgtgcgcactgccagcttcagcaccgcggacagtgccttcgcccccgcctggcggcgcgcgccaccgccgcctcagcactgaaggcgcgctgacgtcactcgccggtcccccgcaaactccccttcccggccaccttggtcgcgtccgcgccgccgccggcccagccggaccgcaccacgcgaggcgcgagataggggggcacgggcgcgaccatctgcgctgcggcgccggcgactcagcgctgcctcagtctgcggtgggcagcggaggagtcgtgtcgtgcctgagagcgcagggatctatttccggtgaattcgccaccatggctgagccccgacaggagttcgaggtaatggaggatcacgcagggacgtatggtctgggagacaggaaggatcaaggcggctatacgatgcaccaggatcaggagggcgataccgatgcgggcctcaaagagtccccgcttcaaacaccaactgaggatgggagtgaggagccaggaagtgagacaagcgacgcgaaatcaacccctactgccgaagcggaggaggccgggatcggagatacaccatctctcgaagacgaagctgctggccacgtgacgcaagcacgaatggtgtccaaaagcaaagacggtacaggttctgacgacaaaaaggcgaagggggcagatgggaaaactaaaatcgccacgccccggggtgcggcgccgcctgggcagaaagggcaagcaaatgcgacgcgaatacctgccaagacgcctccggctcctaagaccccaccatcatctggtgaaccgcctaaaagcggggatcgaagcggttattcatcaccgggtagtccgggtacgccaggctctaggagcagaactccttcactgcccacgccccccacgcgcgaacctaagaaagtggcagtggtgcgaacacccccaaaaagcccctcaagtgcaaaatcacggctccagactgcacccgtaccgatgcccgatctcaaaaacgtgaaatctaagataggtagtacagagaatctgaagcatcaaccgggaggtggaaaggtgcagattatcaataagaaacttgacctgagtaacgttcaatccaagtgtggatcaaaagataatatcaagcacgtccctggaggcggttcagtgcagatcgtttacaaacctgttgatcttagcaaggtgacttccaagtgcgggtctctgggcaacattcatcacaaacctggtggagggcaagttgaggtcaaaagcgaaaagctcgacttcaaagatcgagttcagagcaagataggcagccttgataatattacccatgtccccggcggagggaacaagaagattgagactcataagttgacgttcagagaaaatgctaaagcgaaaacggatcatggcgcagaaatagtttataaatctcctgtggtcagtggtgacacttcacccaggcacctctcaaacgtgtcatcaacgggctcaatcgacatggtggattctccccaactcgcaacacttgctgatgaggtaagtgccagcctcgcaaagcaaggactctaaaattcgctcgagactagttctagagcggccgcggatcccgcccctctccctcccccccccctaacgttactggccgaagccgcttggaataaggccggtgtgcgtttgtctatatgttattttccaccatattgccgtcttttggcaatgtgagggcccggaaacctggccctgtcttcttgacgagcattcctaggggtctttcccctctcgccaaaggaatgcaaggtctgttgaatgtcgtgaaggaagcagttcctctggaagcttcttgaagacaaacaacgtctgtagcgaccctttgcaggcagcggaaccccccacctggcgacaggtgcctctgcggccaaaagccacgtgtataagatacacctgcaaaggcggcacaaccccagtgccacgttgtgagttggatagttgtggaaagagtcaaatggctctcctcaagcgtattcaacaaggggctgaaggatgcccagaaggtaccccattgtatgggatctgatctggggcctcggtgcacatgctttacatgtgtttagtcgaggttaaaaaaacgtctaggccccccgaaccacggggacgtggttttcctttgaaaaacacgatgataagcttgccacaacccgtaccaaagatggatagatccggaaagcctgaactcaccgcgacgtctgtcgagaagtttctgatcgaaaagttcgacagcgtctccgacctgatgcagctctcggagggcgaagaatctcgtgctttcagcttcgatgtaggagggcgtggatatgtcctgcgggtaaatagctgcgccgatggtttctacaaagatcgttatgtttatcggcactttgcatcggccgcgctcccgattccggaagtgcttgacattggggaattcagcgagagcctgacctattgcatctcccgccgtgcacagggtgtcacgttgcaagacctgcctgaaaccgaactgcccgctgttctgcagccggtcgcggaggccatggatgcgatcgctgcggccgatcttagccagacgagcgggttcggcccattcggaccgcaaggaatcggtcaatacactacatggcgtgatttcatatgcgcgattgctgatccccatgtgtatcactggcaaactgtgatggacgacaccgtcagtgcgtccgtcgcgcaggctctcgatgagctgatgctttgggccgaggactgccccgaagtccggcacctcgtgcacgcggatttcggctccaacaatgtcctgacggacaatggccgcataacagcggtcattgactggagcgaggcgatgttcggggattcccaatacgaggtcgccaacatcttcttctggaggccgtggttggcttgtatggagcagcagacgcgctacttcgagcggaggcatccggagcttgcaggatcgccgcggctccgggcgtatatgctccgcattggtcttgaccaactctatcagagcttggttgacggcaatttcgatgatgcagcttgggcgcagggtcgatgcgacgcaatcgtccgatccggagccgggactgtcgggcgtacacaaatcgcccgcagaagcgcggccgtctggaccgatggctgtgtagaagtactcgccgatagtggaaaccgacgccccagcactcgtccgagggcaaaggaatagacgcgtctggaacaatcaacctctggattacaaaatttgtgaaagattgactggtattcttaactatgttgctccttttacgctatgtggatacgctgctttaatgcctttgtatcatgctattgcttcccgtatggctttcattttctcctccttgtataaatcctggttgctgtctctttatgaggagttgtggcccgttgtcaggcaacgtggcgtggtgtgcactgtgtttgctgacgcaacccccactggttggggcattgccaccacctgtcagctcctttccgggactttcgctttccccctccctattgccacggcggaactcatcgccgcctgccttgcccgctgctggacaggggctcggctgttgggcactgacaattccgtggtgttgtcggggaagctgacgtcctttccatggctgctcgcctgtgttgccacctggattctgcgcgggacgtccttctgctacgtcccttcggccctcaatccagcggaccttccttcccgcggcctgctgccggctctgcggcctcttccgcgtcttcgccttcgccctcagacgagtcggatctccctttgggccgcctccccgcctggaattaattctgcagtcgagacctagaaaaacatggagcaatcacaagtagcaatacagcagctaccaatgctgattgtgcctggctagaagcacaagaggaggaggaggtgggttttccagtcacacctcaggtacctttaagaccaatgacttacaaggcagctgtagatcttagccactttttaaaagaaaagaggggactggaagggctaattcactcccaacgaagacaagatatccttgatctgtggatctaccacacacaaggctacttccctgattagcagaactacacaccagggccaggggtcagatatccactgacctttggatggtgctacaagctagtaccagttgagccagataaggtagaagaggccaataaaggagagaacaccagcttgttacaccctgtgagcctgcatgggatggatgacccggagagagaagtgttagagtggaggtttgacagccgcctagcatttcatcacgtggcccgagagctgcatccggagtacttcaagaactgctgatatcgagcttgctacaagggactttccgctggggactttccagggaggcgtggcctgggcgggactggggagtggcgagccctcagatcctgcatataagcagctgctttttgcctgtactgggtctctctggttagaccagatctgagcctgggagctctctggctaactagggaacccactgcttaagcctcaataaagcttgccttgagtgcttcaagtagtgtgtgcccgtctgttgtgtgactctggtaactagagatccctcagacccttttagtcagtgtggaaaatctctagcagtagtagttcatgtcatcttattattcagtatttataacttgcaaagaaatgaatatcagagagtgagaggccttgacattgctagcgtttaccgtcgacctctagctagagcttggcgtaatcatggtcatagctgtttcctgtgtgaaattgttatccgctcacaattccacacaacatacgagccggaagcataaagtgtaaagcctggggtgcctaatgagtgagctaactcacattaattgcgttgcgctcactgcccgctttccagtcgggaaacctgtcgtgccagctgcattaatgaatcggccaacgcgcggggagaggcggtttgcgtattgggcgctcttccgcttcctcgctcactgactcgctgcgctcggtcgttcggctgcggcgagcggtatcagctcactcaaaggcggtaatacggttatccacagaatcaggggataacgcaggaaagaacatgtgagcaaaaggccagcaaaaggccaggaaccgtaaaaaggccgcgttgctggcgtttttccataggctccgcccccctgacgagcatcacaaaaatcgacgctcaagtcagaggtggcgaaacccgacaggactataaagataccaggcgtttccccctggaagctccctcgtgcgctctcctgttccgaccctgccgcttaccggatacctgtccgcctttctcccttcgggaagcgtggcgctttctcatagctcacgctgtaggtatctcagttcggtgtaggtcgttcgctccaagctgggctgtgtgcacgaaccccccgttcagcccgaccgctgcgccttatccggtaactatcgtcttgagtccaacccggtaagacacgacttatcgccactggcagcagccactggtaacaggattagcagagcgaggtatgtaggcggtgctacagagttcttgaagtggtggcctaactacggctacactagaagaacagtatttggtatctgcgctctgctgaagccagttaccttcggaaaaagagttggtagctcttgatccggcaaacaaaccaccgctggtagcggtggtttttttgtttgcaagcagcagattacgcgcagaaaaaaaggatctcaagaagatcctttgatcttttctacggggtctgacgctcagtggaacgaaaactcacgttaagggattttggtcatgagattatcaaaaaggatcttcacctagatccttttaaattaaaaatgaagttttaaatcaatctaaagtatatatgagtaaacttggtctgacagttaccaatgcttaatcagtgaggcacctatctcagcgatctgtctatttcgttcatccatagttgcctgactccccgtcgtgtagataactacgatacgggagggcttaccatctggccccagtgctgcaatgataccgcgagacccacgctcaccggctccagatttatcagcaataaaccagccagccggaagggccgagcgcagaagtggtcctgcaactttatccgcctccatccagtctattaattgttgccgggaagctagagtaagtagttcgccagttaatagtttgcgcaacgttgttgccattgctacaggcatcgtggtgtcacgctcgtcgtttggtatggcttcattcagctccggttcccaacgatcaaggcgagttacatgatcccccatgttgtgcaaaaaagcggttagctccttcggtcctccgatcgttgtcagaagtaagttggccgcagtgttatcactcatggttatggcagcactgcataattctcttactgtcatgccatccgtaagatgcttttctgtgactggtgagtactcaaccaagtcattctgagaatagtgtatgcggcgaccgagttgctcttgcccggcgtcaatacgggataataccgcgccacatagcagaactttaaaagtgctcatcattggaaaacgttcttcggggcgaaaactctcaaggatcttaccgctgttgagatccagttcgatgtaacccactcgtgcacccaactgatcttcagcatcttttactttcaccagcgtttctgggtgagcaaaaacaggaaggcaaaatgccgcaaaaaagggaataagggcgacacggaaatgttgaatactcatactcttcctttttcaatattattgaagcatttatcagggttattgtctcatgagcggatacatatttgaatgtatttagaaaaataaacaaataggggttccgcgcacatttccccgaaaagtgccacctgacgtcgacggatcgggagatcaacttgtttattgcagcttataatggttacaaataaagcaatagcatcacaaatttcacaaataaagcatttttttcactgcattctagttgtggtttgtccaaactcatcaatgtatcttatcatgtctggatcaactggataactcaagctaaccaaaatcatcccaaacttcccaccccataccctattaccactgccaattacctgtggtttcatttactctaaacctgtgattcctctgaattattttcattttaaagaaattgtatttgttaaatatgtactacaaacttagtagt

SEQ ID NO: 76 - DNA, 10350 bp, Artificial Sequence
  Synthetic
  misc_feature (1)..(635): LTR
  misc_feature (636)..(653): PBS
  misc_feature (685)..(822): Packaging\signal
  misc_feature (1303)..(1536): RRE
  misc_feature (2028)..(2151): cPPT
  misc_feature (2185)..(2668): hSynapsin promoter
  misc_feature (2681)..(3916): hTau-412 (1N4R) WT
  misc_feature (3917)..(4630): eGFP
  misc_feature (4640)..(4671): MCS
  misc_feature (4672)..(5270): IRES
  misc_feature (5271)..(6305): HygR
  misc_feature (6319)..(6910): WPRE
  misc_feature (7113)..(7749): LTR
  misc_feature (8218)..(8891): pUC\origin
  misc_feature (9036)..(10032): AmpR
tggaagggctaattcactcccaaagaagacaagatatccttgatctgtggatctaccacacacaaggctacttccctgattagcagaactacacaccagggccaggggtcagatatccactgacctttggatggtgctacaagctagtaccagttgagccagataaggtagaagaggccaataaaggagagaacaccagcttgttacaccctgtgagcctgcatgggatggatgacccggagagagaagtgttagagtggaggtttgacagccgcctagcatttcatcacgtggcccgagagctgcatccggagtacttcaagaactgctgatatcgagcttgctacaagggactttccgctggggactttccagggaggcgtggcctgggcgggactggggagtggcgagccctcagatcctgcatataagcagctgctttttgcctgtactgggtctctctggttagaccagatctgagcctgggagctctctggctaactagggaacccactgcttaagcctcaataaagcttgccttgagtgcttcaagtagtgtgtgcccgtctgttgtgtgactctggtaactagagatccctcagacccttttagtcagtgtggaaaatctctagcagtggcgcccgaacagggacttgaaagcgaaagggaaaccagaggagctctctcgacgcaggactcggcttgctgaagcgcgcacggcaagaggcgaggggcggcgactggtgagtacgccaaaaattttgactagcggaggctagaaggagagagatgggtgcgagagcgtcagtattaagcgggggagaattagatcgcgatgggaaaaaattcggttaaggccagggggaaagaaaaaatataaattaaaacatatagtatgggcaagcagggagctagaacgattcgcagttaatcctggcctgttagaaacatcagaaggctgtagacaaatactgggacagctacaaccatcccttcagacaggatcagaagaacttagatcattatataatacagtagcaaccctctattgtgtgcatcaaaggatagagataaaagacaccaaggaagctttagacaagatagaggaagagcaaaacaaaagtaagaccaccgcacagcaagcggccggccgctgatcttcagacctggaggaggagatatgagggacaattggagaagtgaattatataaatataaagtagtaaaaattgaaccattaggagtagcacccaccaaggcaaagagaagagtggtgcagagagaaaaaagagcagtgggaataggagctttgttccttgggttcttgggagcagcaggaagcactatgggcgcagcgtcaatgacgctgacggtacaggccagacaattattgtctggtatagtgcagcagcagaacaatttgctgagggctattgaggcgcaacagcatctgttgcaactcacagtctggggcatcaagcagctccaggcaagaatcctggctgtggaaagatacctaaaggatcaacagctcctggggatttggggttgctctggaaaactcatttgcaccactgctgtgccttggaatgctagttggagtaataaatctctggaacagatttggaatcacacgacctggatggagtgggacagagaaattaacaattacacaagcttaatacactccttaattgaagaatcgcaaaaccagcaagaaaagaatgaacaagaattattggaattagataaatgggcaagtttgtggaattggtttaacataacaaattggctgtggtatataaaattattcataatgatagtaggaggcttggtaggtttaagaatagtttttgctgtactttctatagtgaatagagttaggcagggatattcaccattatcgtttcagacccacctcccaaccccgaggggacccgacaggcccgaaggaatagaagaagaaggtggagagagagacagagacagatccattcgattagtgaacggatctcgacggtatcgcctttaaaagaaaaggggggattggggggtacagtgcaggggaaagaatagtagacataatagcaacagacatacaaactaaagaattacaaaaacaaattacaaaaattcaaaattttcgggtttattacagggacagcagagatccagtttatcgatctgcagagggccctgcgtatgagtgcaagtgggttttaggaccaggatgaggcggggtgggggtgcctacctgacgaccgaccccgacccactggacaagcacccaacccccattccccaaattgcgcatcccctatcagagagggggaggggaaacaggatgcggcgaggcgcgtgcgcactgccagcttcagcaccgcggacagtgccttcgcccccgcctggcggcgcgcgccaccgccgcctcagcactgaaggcgcgctgacgtcactcgccggtcccccgcaaactccccttcccggccaccttggtcgcgtccgcgccgccgccggcccagccggaccgcaccacgcgaggcgcgagataggggggcacgggcgcgaccatctgcgctgcggcgccggcgactcagcgctgcctcagtctgcggtgggcagcggaggagtcgtgtcgtgcctgagagcgcagggatctatttccggtgaattcgccaccatggctgagccccgacaggagttcgaggtaatggaggatcacgcagggacgtatggtctgggagacaggaaggatcaaggcggctatacgatgcaccaggatcaggagggcgataccgatgcgggcctcaaagagtccccgcttcaaacaccaactgaggatgggagtgaggagccaggaagtgagacaagcgacgcgaaatcaacccctactgccgaagcggaggaggccgggatcggagatacaccatctctcgaagacgaagctgctggccacgtgacgcaagcacgaatggtgtccaaaagcaaagacggtacaggttctgacgacaaaaaggcgaagggggcagatgggaaaactaaaatcgccacgccccggggtgcggcgccgcctgggcagaaagggcaagcaaatgcgacgcgaatacctgccaagacgcctccggctcctaagaccccaccatcatctggtgaaccgcctaaaagcggggatcgaagcggttattcatcaccgggtagtccgggtacgccaggctctaggagcagaactccttcactgcccacgccccccacgcgcgaacctaagaaagtggcagtggtgcgaacacccccaaaaagcccctcaagtgcaaaatcacggctccagactgcacccgtaccgatgcccgatctcaaaaacgtgaaatctaagataggtagtacagagaatctgaagcatcaaccgggaggtggaaaggtgcagattatcaataagaaacttgacctgagtaacgttcaatccaagtgtggatcaaaagataatatcaagcacgtccctggaggcggttcagtgcagatcgtttacaaacctgttgatcttagcaaggtgacttccaagtgcgggtctctgggcaacattcatcacaaacctggtggagggcaagttgaggtcaaaagcgaaaagctcgacttcaaagatcgagttcagagcaagataggcagccttgataatattacccatgtccccggcggagggaacaagaagattgagactcataagttgacgttcagagaaaatgctaaagcgaaaacggatcatggcgcagaaatagtttataaatctcctgtggtcagtggtgacacttcacccaggcacctctcaaacgtgtcatcaacgggctcaatcgacatggtggattctccccaactcgcaacacttgctgatgaggtaagtgccagcctcgcaaagcaaggactcgtgagcaagggcgaggagctgttcaccggggtggtgcccatcctggtcgagctggacggcgacgtaaacggccacaagttcagcgtgtccggcgagggcgagggcgatgccacctacggcaagctgaccctgaagttcatctgcaccaccggcaagctgcccgtgccctggcccaccctcgtgaccaccctgacctacggcgtgcagtgcttcagccgctaccccgaccacatgaagcagcacgacttcttcaagtccgccatgcccgaaggctacgtccaggagcgcaccatcttcttcaaggacgacggcaactacaagacccgcgccgaggtgaagttcgagggcgacaccctggtgaaccgcatcgagctgaagggcatcgacttcaaggaggacggcaacatcctggggcacaagctggagtacaactacaacagccacaacgtctatatcatggccgacaagcagaagaacggcatcaaggtgaacttcaagatccgccacaacatcgaggacggcagcgtgcagctcgccgaccactaccagcagaacacccccatcggcgacggccccgtgctgctgcccgacaaccactacctgagcacccagtccgccctgagcaaagaccccaacgagaagcgcgatcacatggtcctgctggagttcgtgaccgccgccgggatcactctcggcatggacgagctgtacaagtgaaattcgctcgagactagttctagagcggccgcggatcccgcccctctccctcccccccccctaacgttactggccgaagccgcttggaataaggccggtgtgcgtttgtctatatgttattttccaccatattgccgtcttttggcaatgtgagggcccggaaacctggccctgtcttcttgacgagcattcctaggggtctttcccctctcgccaaaggaatgcaaggtctgttgaatgtcgtgaaggaagcagttcctctggaagcttcttgaagacaaacaacgtctgtagcgaccctttgcaggcagcggaaccccccacctggcgacaggtgcctctgcggccaaaagccacgtgtataagatacacctgcaaaggcggcacaaccccagtgccacgttgtgagttggatagttgtggaaagagtcaaatggctctcctcaagcgtattcaacaaggggctgaaggatgcccagaaggtaccccattgtatgggatctgatctggggcctcggtgcacatgctttacatgtgtttagtcgaggttaaaaaaacgtctaggccccccgaaccacggggacgtggttttcctttgaaaaacacgatgataagcttgccacaacccgtaccaaagatggatagatccggaaagcctgaactcaccgcgacgtctgtcgagaagtttctgatcgaaaagttcgacagcgtctccgacctgatgcagctctcggagggcgaagaatctcgtgctttcagcttcgatgtaggagggcgtggatatgtcctgcgggtaaatagctgcgccgatggtttctacaaagatcgttatgtttatcggcactttgcatcggccgcgctcccgattccggaagtgcttgacattggggaattcagcgagagcctgacctattgcatctcccgccgtgcacagggtgtcacgttgcaagacctgcctgaaaccgaactgcccgctgttctgcagccggtcgcggaggccatggatgcgatcgctgcggccgatcttagccagacgagcgggttcggcccattcggaccgcaaggaatcggtcaatacactacatggcgtgatttcatatgcgcgattgctgatccccatgtgtatcactggcaaactgtgatggacgacaccgtcagtgcgtccgtcgcgcaggctctcgatgagctgatgctttgggccgaggactgccccgaagtccggcacctcgtgcacgcggatttcggctccaacaatgtcctgacggacaatggccgcataacagcggtcattgactggagcgaggcgatgttcggggattcccaatacgaggtcgccaacatcttcttctggaggccgtggttggcttgtatggagcagcagacgcgctacttcgagcggaggcatccggagcttgcaggatcgccgcggctccgggcgtatatgctccgcattggtcttgaccaactctatcagagcttggttgacggcaatttcgatgatgcagcttgggcgcagggtcgatgcgacgcaatcgtccgatccggagccgggactgtcgggcgtacacaaatcgcccgcagaagcgcggccgtctggaccgatggctgtgtagaagtactcgccgatagtggaaaccgacgccccagcactcgtccgagggcaaaggaatagacgcgtctggaacaatcaacctctggattacaaaatttgtgaaagattgactggtattcttaactatgttgctccttttacgctatgtggatacgctgctttaatgcctttgtatcatgctattgcttcccgtatggctttcattttctcctccttgtataaatcctggttgctgtctctttatgaggagttgtggcccgttgtcaggcaacgtggcgtggtgtgcactgtgtttgctgacgcaacccccactggttggggcattgccaccacctgtcagctcctttccgggactttcgctttccccctccctattgccacggcggaactcatcgccgcctgccttgcccgctgctggacaggggctcggctgttgggcactgacaattccgtggtgttgtcggggaagctgacgtcctttccatggctgctcgcctgtgttgccacctggattctgcgcgggacgtccttctgctacgtcccttcggccctcaatccagcggaccttccttcccgcggcctgctgccggctctgcggcctcttccgcgtcttcgccttcgccctcagacgagtcggatctccctttgggccgcctccccgcctggaattaattctgcagtcgagacctagaaaaacatggagcaatcacaagtagcaatacagcagctaccaatgctgattgtgcctggctagaagcacaagaggaggaggaggtgggttttccagtcacacctcaggtacctttaagaccaatgacttacaaggcagctgtagatcttagccactttttaaaagaaaagaggggactggaagggctaattcactcccaacgaagacaagatatccttgatctgtggatctaccacacacaaggctacttccctgattagcagaactacacaccagggccaggggtcagatatccactgacctttggatggtgctacaagctagtaccagttgagccagataaggtagaagaggccaataaaggagagaacaccagcttgttacaccctgtgagcctgcatgggatggatgacccggagagagaagtgttagagtggaggtttgacagccgcctagcatttcatcacgtggcccgagagctgcatccggagtacttcaagaactgctgatatcgagcttgctacaagggactttccgctggggactttccagggaggcgtggcctgggcgggactggggagtggcgagccctcagatcctgcatataagcagctgctttttgcctgtactgggtctctctggttagaccagatctgagcctgggagctctctggctaactagggaacccactgcttaagcctcaataaagcttgccttgagtgcttcaagtagtgtgtgcccgtctgttgtgtgactctggtaactagagatccctcagacccttttagtcagtgtggaaaatctctagcagtagtagttcatgtcatcttattattcagtatttataacttgcaaagaaatgaatatcagagagtgagaggccttgacattgctagcgtttaccgtcgacctctagctagagcttggcgtaatcatggtcatagctgtttcctgtgtgaaattgttatccgctcacaattccacacaacatacgagccggaagcataaagtgtaaagcctggggtgcctaatgagtgagctaactcacattaattgcgttgcgctcactgcccgctttccagtcgggaaacctgtcgtgccagctgcattaatgaatcggccaacgcgcggggagaggcggtttgcgtattgggcgctcttccgcttcctcgctcactgactcgctgcgctcggtcgttcggctgcggcgagcggtatcagctcactcaaaggcggtaatacggttatccacagaatcaggggataacgcaggaaagaacatgtgagcaaaaggccagcaaaaggccaggaaccgtaaaaaggccgcgttgctggcgtttttccataggctccgcccccctgacgagcatcacaaaaatcgacgctcaagtcagaggtggcgaaacccgacaggactataaagataccaggcgtttccccctggaagctccctcgtgcgctctcctgttccgaccctgccgcttaccggatacctgtccgcctttctcccttcgggaagcgtggcgctttctcatagctcacgctgtaggtatctcagttcggtgtaggtcgttcgctccaagctgggctgtgtgcacgaaccccccgttcagcccgaccgctgcgccttatccggtaactatcgtcttgagtccaacccggtaagacacgacttatcgccactggcagcagccactggtaacaggattagcagagcgaggtatgtaggcggtgctacagagttcttgaagtggtggcctaactacggctacactagaagaacagtatttggtatctgcgctctgctgaagccagttaccttcggaaaaagagttggtagctcttgatccggcaaacaaaccaccgctggtagcggtggtttttttgtttgcaagcagcagattacgcgcagaaaaaaaggatctcaagaagatcctttgatcttttctacggggtctgacgctcagtggaacgaaaactcacgttaagggattttggtcatgagattatcaaaaaggatcttcacctagatccttttaaattaaaaatgaagttttaaatcaatctaaagtatatatgagtaaacttggtctgacagttaccaatgcttaatcagtgaggcacctatctcagcgatctgtctatttcgttcatccatagttgcctgactccccgtcgtgtagataactacgatacgggagggcttaccatctggccccagtgctgcaatgataccgcgagacccacgctcaccggctccagatttatcagcaataaaccagccagccggaagggccgagcgcagaagtggtcctgcaactttatccgcctccatccagtctattaattgttgccgggaagctagagtaagtagttcgccagttaatagtttgcgcaacgttgttgccattgctacaggcatcgtggtgtcacgctcgtcgtttggtatggcttcattcagctccggttcccaacgatcaaggcgagttacatgatcccccatgttgtgcaaaaaagcggttagctccttcggtcctccgatcgttgtcagaagtaagttggccgcagtgttatcactcatggttatggcagcactgcataattctcttactgtcatgccatccgtaagatgcttttctgtgactggtgagtactcaaccaagtcattctgagaatagtgtatgcggcgaccgagttgctcttgcccggcgtcaatacgggataataccgcgccacatagcagaactttaaaagtgctcatcattggaaaacgttcttcggggcgaaaactctcaaggatcttaccgctgttgagatccagttcgatgtaacccactcgtgcacccaactgatcttcagcatcttttactttcaccagcgtttctgggtgagcaaaaacaggaaggcaaaatgccgcaaaaaagggaataagggcgacacggaaatgttgaatactcatactcttcctttttcaatattattgaagcatttatcagggttattgtctcatgagcggatacatatttgaatgtatttagaaaaataaacaaataggggttccgcgcacatttccccgaaaagtgccacctgacgtcgacggatcgggagatcaacttgtttattgcagcttataatggttacaaataaagcaatagcatcacaaatttcacaaataaagcatttttttcactgcattctagttgtggtttgtccaaactcatcaatgtatcttatcatgtctggatcaactggataactcaagctaaccaaaatcatcccaaacttcccaccccataccctattaccactgccaattacctgtggtttcatttactctaaacctgtgattcctctgaattattttcattttaaagaaattgtatttgttaaatatgtactacaaacttagtagt

SEQ ID NO: 77 - DNA, 10350 bp, Artificial Sequence
  Synthetic
  misc_feature (1)..(635): LTR
  misc_feature (636)..(653): PBS
  misc_feature (685)..(822): Packaging\signal
  misc_feature (1303)..(1536): RRE
  misc_feature (2028)..(2151): cPPT
  misc_feature (2185)..(2668): hSynapsin promoter
  misc_feature (2681)..(3397): eGFP
  misc_feature (3398)..(4633): hTau-412 (1NR4) WT
  misc_feature (4640)..(4671): MCS
  misc_feature (4672)..(5270): IRES
  misc_feature (5271)..(6305): HygR
  misc_feature (6319)..(6910): WPRE
  misc_feature (7113)..(7749): LTR
  misc_feature (8218)..(8891): pUC\origin
  misc_feature (9036)..(10032): AmpR
tggaagggctaattcactcccaaagaagacaagatatccttgatctgtggatctaccacacacaaggctacttccctgattagcagaactacacaccagggccaggggtcagatatccactgacctttggatggtgctacaagctagtaccagttgagccagataaggtagaagaggccaataaaggagagaacaccagcttgttacaccctgtgagcctgcatgggatggatgacccggagagagaagtgttagagtggaggtttgacagccgcctagcatttcatcacgtggcccgagagctgcatccggagtacttcaagaactgctgatatcgagcttgctacaagggactttccgctggggactttccagggaggcgtggcctgggcgggactggggagtggcgagccctcagatcctgcatataagcagctgctttttgcctgtactgggtctctctggttagaccagatctgagcctgggagctctctggctaactagggaacccactgcttaagcctcaataaagcttgccttgagtgcttcaagtagtgtgtgcccgtctgttgtgtgactctggtaactagagatccctcagacccttttagtcagtgtggaaaatctctagcagtggcgcccgaacagggacttgaaagcgaaagggaaaccagaggagctctctcgacgcaggactcggcttgctgaagcgcgcacggcaagaggcgaggggcggcgactggtgagtacgccaaaaattttgactagcggaggctagaaggagagagatgggtgcgagagcgtcagtattaagcgggggagaattagatcgcgatgggaaaaaattcggttaaggccagggggaaagaaaaaatataaattaaaacatatagtatgggcaagcagggagctagaacgattcgcagttaatcctggcctgttagaaacatcagaaggctgtagacaaatactgggacagctacaaccatcccttcagacaggatcagaagaacttagatcattatataatacagtagcaaccctctattgtgtgcatcaaaggatagagataaaagacaccaaggaagctttagacaagatagaggaagagcaaaacaaaagtaagaccaccgcacagcaagcggccggccgctgatcttcagacctggaggaggagatatgagggacaattggagaagtgaattatataaatataaagtagtaaaaattgaaccattaggagtagcacccaccaaggcaaagagaagagtggtgcagagagaaaaaagagcagtgggaataggagctttgttccttgggttcttgggagcagcaggaagcactatgggcgcagcgtcaatgacgctgacggtacaggccagacaattattgtctggtatagtgcagcagcagaacaatttgctgagggctattgaggcgcaacagcatctgttgcaactcacagtctggggcatcaagcagctccaggcaagaatcctggctgtggaaagatacctaaaggatcaacagctcctggggatttggggttgctctggaaaactcatttgcaccactgctgtgccttggaatgctagttggagtaataaatctctggaacagatttggaatcacacgacctggatggagtgggacagagaaattaacaattacacaagcttaatacactccttaattgaagaatcgcaaaaccagcaagaaaagaatgaacaagaattattggaattagataaatgggcaagtttgtggaattggtttaacataacaaattggctgtggtatataaaattattcataatgatagtaggaggcttggtaggtttaagaatagtttttgctgtactttctatagtgaatagagttaggcagggatattcaccattatcgtttcagacccacctcccaaccccgaggggacccgacaggcccgaaggaatagaagaagaaggtggagagagagacagagacagatccattcgattagtgaacggatctcgacggtatcgcctttaaaagaaaaggggggattggggggtacagtgcaggggaaagaatagtagacataatagcaacagacatacaaactaaagaattacaaaaacaaattacaaaaattcaaaattttcgggtttattacagggacagcagagatccagtttatcgatctgcagagggccctgcgtatgagtgcaagtgggttttaggaccaggatgaggcggggtgggggtgcctacctgacgaccgaccccgacccactggacaagcacccaacccccattccccaaattgcgcatcccctatcagagagggggaggggaaacaggatgcggcgaggcgcgtgcgcactgccagcttcagcaccgcggacagtgccttcgcccccgcctggcggcgcgcgccaccgccgcctcagcactgaaggcgcgctgacgtcactcgccggtcccccgcaaactccccttcccggccaccttggtcgcgtccgcgccgccgccggcccagccggaccgcaccacgcgaggcgcgagataggggggcacgggcgcgaccatctgcgctgcggcgccggcgactcagcgctgcctcagtctgcggtgggcagcggaggagtcgtgtcgtgcctgagagcgcagggatctatttccggtgaattcgccaccatggtgagcaagggcgaggagctgttcaccggggtggtgcccatcctggtcgagctggacggcgacgtaaacggccacaagttcagcgtgtccggcgagggcgagggcgatgccacctacggcaagctgaccctgaagttcatctgcaccaccggcaagctgcccgtgccctggcccaccctcgtgaccaccctgacctacggcgtgcagtgcttcagccgctaccccgaccacatgaagcagcacgacttcttcaagtccgccatgcccgaaggctacgtccaggagcgcaccatcttcttcaaggacgacggcaactacaagacccgcgccgaggtgaagttcgagggcgacaccctggtgaaccgcatcgagctgaagggcatcgacttcaaggaggacggcaacatcctggggcacaagctggagtacaactacaacagccacaacgtctatatcatggccgacaagcagaagaacggcatcaaggtgaacttcaagatccgccacaacatcgaggacggcagcgtgcagctcgccgaccactaccagcagaacacccccatcggcgacggccccgtgctgctgcccgacaaccactacctgagcacccagtccgccctgagcaaagaccccaacgagaagcgcgatcacatggtcctgctggagttcgtgaccgccgccgggatcactctcggcatggacgagctgtacaaggctgagccccgacaggagttcgaggtaatggaggatcacgcagggacgtatggtctgggagacaggaaggatcaaggcggctatacgatgcaccaggatcaggagggcgataccgatgcgggcctcaaagagtccccgcttcaaacaccaactgaggatgggagtgaggagccaggaagtgagacaagcgacgcgaaatcaacccctactgccgaagcggaggaggccgggatcggagatacaccatctctcgaagacgaagctgctggccacgtgacgcaagcacgaatggtgtccaaaagcaaagacggtacaggttctgacgacaaaaaggcgaagggggcagatgggaaaactaaaatcgccacgccccggggtgcggcgccgcctgggcagaaagggcaagcaaatgcgacgcgaatacctgccaagacgcctccggctcctaagaccccaccatcatctggtgaaccgcctaaaagcggggatcgaagcggttattcatcaccgggtagtccgggtacgccaggctctaggagcagaactccttcactgcccacgccccccacgcgcgaacctaagaaagtggcagtggtgcgaacacccccaaaaagcccctcaagtgcaaaatcacggctccagactgcacccgtaccgatgcccgatctcaaaaacgtgaaatctaagataggtagtacagagaatctgaagcatcaaccgggaggtggaaaggtgcagattatcaataagaaacttgacctgagtaacgttcaatccaagtgtggatcaaaagataatatcaagcacgtccctggaggcggttcagtgcagatcgtttacaaacctgttgatcttagcaaggtgacttccaagtgcgggtctctgggcaacattcatcacaaacctggtggagggcaagttgaggtcaaaagcgaaaagctcgacttcaaagatcgagttcagagcaagataggcagccttgataatattacccatgtccccggcggagggaacaagaagattgagactcataagttgacgttcagagaaaatgctaaagcgaaaacggatcatggcgcagaaatagtttataaatctcctgtggtcagtggtgacacttcacccaggcacctctcaaacgtgtcatcaacgggctcaatcgacatggtggattctccccaactcgcaacacttgctgatgaggtaagtgccagcctcgcaaagcaaggactctaaaattcgctcgagactagttctagagcggccgcggatcccgcccctctccctcccccccccctaacgttactggccgaagccgcttggaataaggccggtgtgcgtttgtctatatgttattttccaccatattgccgtcttttggcaatgtgagggcccggaaacctggccctgtcttcttgacgagcattcctaggggtctttcccctctcgccaaaggaatgcaaggtctgttgaatgtcgtgaaggaagcagttcctctggaagcttcttgaagacaaacaacgtctgtagcgaccctttgcaggcagcggaaccccccacctggcgacaggtgcctctgcggccaaaagccacgtgtataagatacacctgcaaaggcggcacaaccccagtgccacgttgtgagttggatagttgtggaaagagtcaaatggctctcctcaagcgtattcaacaaggggctgaaggatgcccagaaggtaccccattgtatgggatctgatctggggcctcggtgcacatgctttacatgtgtttagtcgaggttaaaaaaacgtctaggccccccgaaccacggggacgtggttttcctttgaaaaacacgatgataagcttgccacaacccgtaccaaagatggatagatccggaaagcctgaactcaccgcgacgtctgtcgagaagtttctgatcgaaaagttcgacagcgtctccgacctgatgcagctctcggagggcgaagaatctcgtgctttcagcttcgatgtaggagggcgtggatatgtcctgcgggtaaatagctgcgccgatggtttctacaaagatcgttatgtttatcggcactttgcatcggccgcgctcccgattccggaagtgcttgacattggggaattcagcgagagcctgacctattgcatctcccgccgtgcacagggtgtcacgttgcaagacctgcctgaaaccgaactgcccgctgttctgcagccggtcgcggaggccatggatgcgatcgctgcggccgatcttagccagacgagcgggttcggcccattcggaccgcaaggaatcggtcaatacactacatggcgtgatttcatatgcgcgattgctgatccccatgtgtatcactggcaaactgtgatggacgacaccgtcagtgcgtccgtcgcgcaggctctcgatgagctgatgctttgggccgaggactgccccgaagtccggcacctcgtgcacgcggatttcggctccaacaatgtcctgacggacaatggccgcataacagcggtcattgactggagcgaggcgatgttcggggattcccaatacgaggtcgccaacatcttcttctggaggccgtggttggcttgtatggagcagcagacgcgctacttcgagcggaggcatccggagcttgcaggatcgccgcggctccgggcgtatatgctccgcattggtcttgaccaactctatcagagcttggttgacggcaatttcgatgatgcagcttgggcgcagggtcgatgcgacgcaatcgtccgatccggagccgggactgtcgggcgtacacaaatcgcccgcagaagcgcggccgtctggaccgatggctgtgtagaagtactcgccgatagtggaaaccgacgccccagcactcgtccgagggcaaaggaatagacgcgtctggaacaatcaacctctggattacaaaatttgtgaaagattgactggtattcttaactatgttgctccttttacgctatgtggatacgctgctttaatgcctttgtatcatgctattgcttcccgtatggctttcattttctcctccttgtataaatcctggttgctgtctctttatgaggagttgtggcccgttgtcaggcaacgtggcgtggtgtgcactgtgtttgctgacgcaacccccactggttggggcattgccaccacctgtcagctcctttccgggactttcgctttccccctccctattgccacggcggaactcatcgccgcctgccttgcccgctgctggacaggggctcggctgttgggcactgacaattccgtggtgttgtcggggaagctgacgtcctttccatggctgctcgcctgtgttgccacctggattctgcgcgggacgtccttctgctacgtcccttcggccctcaatccagcggaccttccttcccgcggcctgctgccggctctgcggcctcttccgcgtcttcgccttcgccctcagacgagtcggatctccctttgggccgcctccccgcctggaattaattctgcagtcgagacctagaaaaacatggagcaatcacaagtagcaatacagcagctaccaatgctgattgtgcctggctagaagcacaagaggaggaggaggtgggttttccagtcacacctcaggtacctttaagaccaatgacttacaaggcagctgtagatcttagccactttttaaaagaaaagaggggactggaagggctaattcactcccaacgaagacaagatatccttgatctgtggatctaccacacacaaggctacttccctgattagcagaactacacaccagggccaggggtcagatatccactgacctttggatggtgctacaagctagtaccagttgagccagataaggtagaagaggccaataaaggagagaacaccagcttgttacaccctgtgagcctgcatgggatggatgacccggagagagaagtgttagagtggaggtttgacagccgcctagcatttcatcacgtggcccgagagctgcatccggagtacttcaagaactgctgatatcgagcttgctacaagggactttccgctggggactttccagggaggcgtggcctgggcgggactggggagtggcgagccctcagatcctgcatataagcagctgctttttgcctgtactgggtctctctggttagaccagatctgagcctgggagctctctggctaactagggaacccactgcttaagcctcaataaagcttgccttgagtgcttcaagtagtgtgtgcccgtctgttgtgtgactctggtaactagagatccctcagacccttttagtcagtgtggaaaatctctagcagtagtagttcatgtcatcttattattcagtatttataacttgcaaagaaatgaatatcagagagtgagaggccttgacattgctagcgtttaccgtcgacctctagctagagcttggcgtaatcatggtcatagctgtttcctgtgtgaaattgttatccgctcacaattccacacaacatacgagccggaagcataaagtgtaaagcctggggtgcctaatgagtgagctaactcacattaattgcgttgcgctcactgcccgctttccagtcgggaaacctgtcgtgccagctgcattaatgaatcggccaacgcgcggggagaggcggtttgcgtattgggcgctcttccgcttcctcgctcactgactcgctgcgctcggtcgttcggctgcggcgagcggtatcagctcactcaaaggcggtaatacggttatccacagaatcaggggataacgcaggaaagaacatgtgagcaaaaggccagcaaaaggccaggaaccgtaaaaaggccgcgttgctggcgtttttccataggctccgcccccctgacgagcatcacaaaaatcgacgctcaagtcagaggtggcgaaacccgacaggactataaagataccaggcgtttccccctggaagctccctcgtgcgctctcctgttccgaccctgccgcttaccggatacctgtccgcctttctcccttcgggaagcgtggcgctttctcatagctcacgctgtaggtatctcagttcggtgtaggtcgttcgctccaagctgggctgtgtgcacgaaccccccgttcagcccgaccgctgcgccttatccggtaactatcgtcttgagtccaacccggtaagacacgacttatcgccactggcagcagccactggtaacaggattagcagagcgaggtatgtaggcggtgctacagagttcttgaagtggtggcctaactacggctacactagaagaacagtatttggtatctgcgctctgctgaagccagttaccttcggaaaaagagttggtagctcttgatccggcaaacaaaccaccgctggtagcggtggtttttttgtttgcaagcagcagattacgcgcagaaaaaaaggatctcaagaagatcctttgatcttttctacggggtctgacgctcagtggaacgaaaactcacgttaagggattttggtcatgagattatcaaaaaggatcttcacctagatccttttaaattaaaaatgaagttttaaatcaatctaaagtatatatgagtaaacttggtctgacagttaccaatgcttaatcagtgaggcacctatctcagcgatctgtctatttcgttcatccatagttgcctgactccccgtcgtgtagataactacgatacgggagggcttaccatctggccccagtgctgcaatgataccgcgagacccacgctcaccggctccagatttatcagcaataaaccagccagccggaagggccgagcgcagaagtggtcctgcaactttatccgcctccatccagtctattaattgttgccgggaagctagagtaagtagttcgccagttaatagtttgcgcaacgttgttgccattgctacaggcatcgtggtgtcacgctcgtcgtttggtatggcttcattcagctccggttcccaacgatcaaggcgagttacatgatcccccatgttgtgcaaaaaagcggttagctccttcggtcctccgatcgttgtcagaagtaagttggccgcagtgttatcactcatggttatggcagcactgcataattctcttactgtcatgccatccgtaagatgcttttctgtgactggtgagtactcaaccaagtcattctgagaatagtgtatgcggcgaccgagttgctcttgcccggcgtcaatacgggataataccgcgccacatagcagaactttaaaagtgctcatcattggaaaacgttcttcggggcgaaaactctcaaggatcttaccgctgttgagatccagttcgatgtaacccactcgtgcacccaactgatcttcagcatcttttactttcaccagcgtttctgggtgagcaaaaacaggaaggcaaaatgccgcaaaaaagggaataagggcgacacggaaatgttgaatactcatactcttcctttttcaatattattgaagcatttatcagggttattgtctcatgagcggatacatatttgaatgtatttagaaaaataaacaaataggggttccgcgcacatttccccgaaaagtgccacctgacgtcgacggatcgggagatcaacttgtttattgcagcttataatggttacaaataaagcaatagcatcacaaatttcacaaataaagcatttttttcactgcattctagttgtggtttgtccaaactcatcaatgtatcttatcatgtctggatcaactggataactcaagctaaccaaaatcatcccaaacttcccaccccataccctattaccactgccaattacctgtggtttcatttactctaaacctgtgattcctctgaattattttcattttaaagaaattgtatttgttaaatatgtactacaaacttagtagt

SEQ ID NO: 78 - DNA, 9636 bp, Artificial Sequence
  Synthetic
  misc_feature (1)..(635): LTR
  misc_feature (636)..(653): PBS
  misc_feature (685)..(822): Packaging\signal
  misc_feature (1303)..(1536): RRE
  misc_feature (2028)..(2151): cPPT
  misc_feature (2185)..(2668): hSynapsin promoter
  misc_feature (2681)..(3919): CoHu hTau-412(1N4R) 3MUT
  misc_feature (3926)..(3957): MCS
  misc_feature (3958)..(4556): IRES
  misc_feature (4557)..(5591): HygR
  misc_feature (5605)..(6196): WPRE
  misc_feature (6399)..(7035): LTR
  misc_feature (7504)..(8177): pUC\origin
  misc_feature (8322)..(9318): AmpR
tggaagggctaattcactcccaaagaagacaagatatccttgatctgtggatctaccacacacaaggctacttccctgattagcagaactacacaccagggccaggggtcagatatccactgacctttggatggtgctacaagctagtaccagttgagccagataaggtagaagaggccaataaaggagagaacaccagcttgttacaccctgtgagcctgcatgggatggatgacccggagagagaagtgttagagtggaggtttgacagccgcctagcatttcatcacgtggcccgagagctgcatccggagtacttcaagaactgctgatatcgagcttgctacaagggactttccgctggggactttccagggaggcgtggcctgggcgggactggggagtggcgagccctcagatcctgcatataagcagctgctttttgcctgtactgggtctctctggttagaccagatctgagcctgggagctctctggctaactagggaacccactgcttaagcctcaataaagcttgccttgagtgcttcaagtagtgtgtgcccgtctgttgtgtgactctggtaactagagatccctcagacccttttagtcagtgtggaaaatctctagcagtggcgcccgaacagggacttgaaagcgaaagggaaaccagaggagctctctcgacgcaggactcggcttgctgaagcgcgcacggcaagaggcgaggggcggcgactggtgagtacgccaaaaattttgactagcggaggctagaaggagagagatgggtgcgagagcgtcagtattaagcgggggagaattagatcgcgatgggaaaaaattcggttaaggccagggggaaagaaaaaatataaattaaaacatatagtatgggcaagcagggagctagaacgattcgcagttaatcctggcctgttagaaacatcagaaggctgtagacaaatactgggacagctacaaccatcccttcagacaggatcagaagaacttagatcattatataatacagtagcaaccctctattgtgtgcatcaaaggatagagataaaagacaccaaggaagctttagacaagatagaggaagagcaaaacaaaagtaagaccaccgcacagcaagcggccggccgctgatcttcagacctggaggaggagatatgagggacaattggagaagtgaattatataaatataaagtagtaaaaattgaaccattaggagtagcacccaccaaggcaaagagaagagtggtgcagagagaaaaaagagcagtgggaataggagctttgttccttgggttcttgggagcagcaggaagcactatgggcgcagcgtcaatgacgctgacggtacaggccagacaattattgtctggtatagtgcagcagcagaacaatttgctgagggctattgaggcgcaacagcatctgttgcaactcacagtctggggcatcaagcagctccaggcaagaatcctggctgtggaaagatacctaaaggatcaacagctcctggggatttggggttgctctggaaaactcatttgcaccactgctgtgccttggaatgctagttggagtaataaatctctggaacagatttggaatcacacgacctggatggagtgggacagagaaattaacaattacacaagcttaatacactccttaattgaagaatcgcaaaaccagcaagaaaagaatgaacaagaattattggaattagataaatgggcaagtttgtggaattggtttaacataacaaattggctgtggtatataaaattattcataatgatagtaggaggcttggtaggtttaagaatagtttttgctgtactttctatagtgaatagagttaggcagggatattcaccattatcgtttcagacccacctcccaaccccgaggggacccgacaggcccgaaggaatagaagaagaaggtggagagagagacagagacagatccattcgattagtgaacggatctcgacggtatcgcctttaaaagaaaaggggggattggggggtacagtgcaggggaaagaatagtagacataatagcaacagacatacaaactaaagaattacaaaaacaaattacaaaaattcaaaattttcgggtttattacagggacagcagagatccagtttatcgatctgcagagggccctgcgtatgagtgcaagtgggttttaggaccaggatgaggcggggtgggggtgcctacctgacgaccgaccccgacccactggacaagcacccaacccccattccccaaattgcgcatcccctatcagagagggggaggggaaacaggatgcggcgaggcgcgtgcgcactgccagcttcagcaccgcggacagtgccttcgcccccgcctggcggcgcgcgccaccgccgcctcagcactgaaggcgcgctgacgtcactcgccggtcccccgcaaactccccttcccggccaccttggtcgcgtccgcgccgccgccggcccagccggaccgcaccacgcgaggcgcgagataggggggcacgggcgcgaccatctgcgctgcggcgccggcgactcagcgctgcctcagtctgcggtgggcagcggaggagtcgtgtcgtgcctgagagcgcagggatctatttccggtgaattcgccaccatggcagagccccggcaggagttcgaggttatggaggatcacgccgggacctatggattgggcgataggaaagatcagggcgggtatactatgcatcaggaccaggaaggcgacacggacgctggtctcaaggaaagcccacttcagacgccgacagaggacgggtctgaggaacctgggagtgaaacttctgacgctaagtctacgcctactgcggaggcggaggaggcaggaataggagacacaccatcacttgaagacgaggcagcaggacacgtaacccaagcgagaatggtttctaagtccaaagatggaaccggatccgatgacaaaaaggccaagggagcagatggcaaaacaaaaataacgacaccgaggggtgcggctccccccggtcaaaagggacaggcaaatgccacgcgcatccctgctaaaacacccccggcgccgaaaacccccccttcatccggagagccacccaagtctggtgatagaagcgggtatagttcccccggtagtccggggactccaggatcacgcagcagaacgccatccctgccaaccccacccactagagagcccaaaaaggtcgcagtcgttcgcactccgccaaaaagcccttcctcagcgaaaagccgcctgcagacggcacctgtccccatgcctgaccttaaaaatgttaaaagcaaaatcggtagtaccgaaaatctcaagcatcagccaggaggggggaaggttcagatcatcaataagaagctggacctgtctaacgtgcagagcaagtgtggaagcaaagataacataaagcacgttttggggggcggaagcgtacagattgtgtataagccggtggacctctcaaaagtaacattcaagtgtgggagtctgggcaacatccatcacaaacccgggggcggtcaggtagaggtgaaaagcgaaaagctcgattttaaggatagggtacagagtaaaattgggtctctggacaacataacacacgtaccaggcggaggcaataagaagatagaaacgcataaactcacgttccgagagaacgctaaagcaaagactgaccacggggctgagattgtatacaagagtccggtcgtctctggggacacttccccccgacacctttctaacgttagttccactggtagtattgacatggtcgacagccctcaacttgccactttggcagacgaggtcagtgctagtcttgcaaagcagggcttgtgaaattcgctcgagactagttctagagcggccgcggatcccgcccctctccctcccccccccctaacgttactggccgaagccgcttggaataaggccggtgtgcgtttgtctatatgttattttccaccatattgccgtcttttggcaatgtgagggcccggaaacctggccctgtcttcttgacgagcattcctaggggtctttcccctctcgccaaaggaatgcaaggtctgttgaatgtcgtgaaggaagcagttcctctggaagcttcttgaagacaaacaacgtctgtagcgaccctttgcaggcagcggaaccccccacctggcgacaggtgcctctgcggccaaaagccacgtgtataagatacacctgcaaaggcggcacaaccccagtgccacgttgtgagttggatagttgtggaaagagtcaaatggctctcctcaagcgtattcaacaaggggctgaaggatgcccagaaggtaccccattgtatgggatctgatctggggcctcggtgcacatgctttacatgtgtttagtcgaggttaaaaaaacgtctaggccccccgaaccacggggacgtggttttcctttgaaaaacacgatgataagcttgccacaacccgtaccaaagatggatagatccggaaagcctgaactcaccgcgacgtctgtcgagaagtttctgatcgaaaagttcgacagcgtctccgacctgatgcagctctcggagggcgaagaatctcgtgctttcagcttcgatgtaggagggcgtggatatgtcctgcgggtaaatagctgcgccgatggtttctacaaagatcgttatgtttatcggcactttgcatcggccgcgctcccgattccggaagtgcttgacattggggaattcagcgagagcctgacctattgcatctcccgccgtgcacagggtgtcacgttgcaagacctgcctgaaaccgaactgcccgctgttctgcagccggtcgcggaggccatggatgcgatcgctgcggccgatcttagccagacgagcgggttcggcccattcggaccgcaaggaatcggtcaatacactacatggcgtgatttcatatgcgcgattgctgatccccatgtgtatcactggcaaactgtgatggacgacaccgtcagtgcgtccgtcgcgcaggctctcgatgagctgatgctttgggccgaggactgccccgaagtccggcacctcgtgcacgcggatttcggctccaacaatgtcctgacggacaatggccgcataacagcggtcattgactggagcgaggcgatgttcggggattcccaatacgaggtcgccaacatcttcttctggaggccgtggttggcttgtatggagcagcagacgcgctacttcgagcggaggcatccggagcttgcaggatcgccgcggctccgggcgtatatgctccgcattggtcttgaccaactctatcagagcttggttgacggcaatttcgatgatgcagcttgggcgcagggtcgatgcgacgcaatcgtccgatccggagccgggactgtcgggcgtacacaaatcgcccgcagaagcgcggccgtctggaccgatggctgtgtagaagtactcgccgatagtggaaaccgacgccccagcactcgtccgagggcaaaggaatagacgcgtctggaacaatcaacctctggattacaaaatttgtgaaagattgactggtattcttaactatgttgctccttttacgctatgtggatacgctgctttaatgcctttgtatcatgctattgcttcccgtatggctttcattttctcctccttgtataaatcctggttgctgtctctttatgaggagttgtggcccgttgtcaggcaacgtggcgtggtgtgcactgtgtttgctgacgcaacccccactggttggggcattgccaccacctgtcagctcctttccgggactttcgctttccccctccctattgccacggcggaactcatcgccgcctgccttgcccgctgctggacaggggctcggctgttgggcactgacaattccgtggtgttgtcggggaagctgacgtcctttccatggctgctcgcctgtgttgccacctggattctgcgcgggacgtccttctgctacgtcccttcggccctcaatccagcggaccttccttcccgcggcctgctgccggctctgcggcctcttccgcgtcttcgccttcgccctcagacgagtcggatctccctttgggccgcctccccgcctggaattaattctgcagtcgagacctagaaaaacatggagcaatcacaagtagcaatacagcagctaccaatgctgattgtgcctggctagaagcacaagaggaggaggaggtgggttttccagtcacacctcaggtacctttaagaccaatgacttacaaggcagctgtagatcttagccactttttaaaagaaaagaggggactggaagggctaattcactcccaacgaagacaagatatccttgatctgtggatctaccacacacaaggctacttccctgattagcagaactacacaccagggccaggggtcagatatccactgacctttggatggtgctacaagctagtaccagttgagccagataaggtagaagaggccaataaaggagagaacaccagcttgttacaccctgtgagcctgcatgggatggatgacccggagagagaagtgttagagtggaggtttgacagccgcctagcatttcatcacgtggcccgagagctgcatccggagtacttcaagaactgctgatatcgagcttgctacaagggactttccgctggggactttccagggaggcgtggcctgggcgggactggggagtggcgagccctcagatcctgcatataagcagctgctttttgcctgtactgggtctctctggttagaccagatctgagcctgggagctctctggctaactagggaacccactgcttaagcctcaataaagcttgccttgagtgcttcaagtagtgtgtgcccgtctgttgtgtgactctggtaactagagatccctcagacccttttagtcagtgtggaaaatctctagcagtagtagttcatgtcatcttattattcagtatttataacttgcaaagaaatgaatatcagagagtgagaggccttgacattgctagcgtttaccgtcgacctctagctagagcttggcgtaatcatggtcatagctgtttcctgtgtgaaattgttatccgctcacaattccacacaacatacgagccggaagcataaagtgtaaagcctggggtgcctaatgagtgagctaactcacattaattgcgttgcgctcactgcccgctttccagtcgggaaacctgtcgtgccagctgcattaatgaatcggccaacgcgcggggagaggcggtttgcgtattgggcgctcttccgcttcctcgctcactgactcgctgcgctcggtcgttcggctgcggcgagcggtatcagctcactcaaaggcggtaatacggttatccacagaatcaggggataacgcaggaaagaacatgtgagcaaaaggccagcaaaaggccaggaaccgtaaaaaggccgcgttgctggcgtttttccataggctccgcccccctgacgagcatcacaaaaatcgacgctcaagtcagaggtggcgaaacccgacaggactataaagataccaggcgtttccccctggaagctccctcgtgcgctctcctgttccgaccctgccgcttaccggatacctgtccgcctttctcccttcgggaagcgtggcgctttctcatagctcacgctgtaggtatctcagttcggtgtaggtcgttcgctccaagctgggctgtgtgcacgaaccccccgttcagcccgaccgctgcgccttatccggtaactatcgtcttgagtccaacccggtaagacacgacttatcgccactggcagcagccactggtaacaggattagcagagcgaggtatgtaggcggtgctacagagttcttgaagtggtggcctaactacggctacactagaagaacagtatttggtatctgcgctctgctgaagccagttaccttcggaaaaagagttggtagctcttgatccggcaaacaaaccaccgctggtagcggtggtttttttgtttgcaagcagcagattacgcgcagaaaaaaaggatctcaagaagatcctttgatcttttctacggggtctgacgctcagtggaacgaaaactcacgttaagggattttggtcatgagattatcaaaaaggatcttcacctagatccttttaaattaaaaatgaagttttaaatcaatctaaagtatatatgagtaaacttggtctgacagttaccaatgcttaatcagtgaggcacctatctcagcgatctgtctatttcgttcatccatagttgcctgactccccgtcgtgtagataactacgatacgggagggcttaccatctggccccagtgctgcaatgataccgcgagacccacgctcaccggctccagatttatcagcaataaaccagccagccggaagggccgagcgcagaagtggtcctgcaactttatccgcctccatccagtctattaattgttgccgggaagctagagtaagtagttcgccagttaatagtttgcgcaacgttgttgccattgctacaggcatcgtggtgtcacgctcgtcgtttggtatggcttcattcagctccggttcccaacgatcaaggcgagttacatgatcccccatgttgtgcaaaaaagcggttagctccttcggtcctccgatcgttgtcagaagtaagttggccgcagtgttatcactcatggttatggcagcactgcataattctcttactgtcatgccatccgtaagatgcttttctgtgactggtgagtactcaaccaagtcattctgagaatagtgtatgcggcgaccgagttgctcttgcccggcgtcaatacgggataataccgcgccacatagcagaactttaaaagtgctcatcattggaaaacgttcttcggggcgaaaactctcaaggatcttaccgctgttgagatccagttcgatgtaacccactcgtgcacccaactgatcttcagcatcttttactttcaccagcgtttctgggtgagcaaaaacaggaaggcaaaatgccgcaaaaaagggaataagggcgacacggaaatgttgaatactcatactcttcctttttcaatattattgaagcatttatcagggttattgtctcatgagcggatacatatttgaatgtatttagaaaaataaacaaataggggttccgcgcacatttccccgaaaagtgccacctgacgtcgacggatcgggagatcaacttgtttattgcagcttataatggttacaaataaagcaatagcatcacaaatttcacaaataaagcatttttttcactgcattctagttgtggtttgtccaaactcatcaatgtatcttatcatgtctggatcaactggataactcaagctaaccaaaatcatcccaaacttcccaccccataccctattaccactgccaattacctgtggtttcatttactctaaacctgtgattcctctgaattattttcattttaaagaaattgtatttgttaaatatgtactacaaacttagtagt

SEQ ID NO: 79 - DNA, 10350 bp, Artificial Sequence
  Synthetic
  misc_feature (1)..(635): LTR
  misc_feature (636)..(653): PBS
  misc_feature (685)..(822): Packaging\signal
  misc_feature (1303)..(1536): RRE
  misc_feature (2028)..(2151): cPPT
  misc_feature (2185)..(2668): hSynapsin promoter
  misc_feature (2681)..(3916): CoHu hTau-412(1N4R) 3MUT
  misc_feature (3917)..(4630): eGFP
  misc_feature (4640)..(4671): MCS
  misc_feature (4672)..(5270): IRES
  misc_feature (5271)..(6305): HygR
  misc_feature (6319)..(6910): WPRE
  misc_feature (7113)..(7749): LTR
  misc_feature (8218)..(8891): pUC\origin
  misc_feature (9036)..(10032): AmpR
tggaagggctaattcactcccaaagaagacaagatatccttgatctgtggatctaccacacacaaggctacttccctgattagcagaactacacaccagggccaggggtcagatatccactgacctttggatggtgctacaagctagtaccagttgagccagataaggtagaagaggccaataaaggagagaacaccagcttgttacaccctgtgagcctgcatgggatggatgacccggagagagaagtgttagagtggaggtttgacagccgcctagcatttcatcacgtggcccgagagctgcatccggagtacttcaagaactgctgatatcgagcttgctacaagggactttccgctggggactttccagggaggcgtggcctgggcgggactggggagtggcgagccctcagatcctgcatataagcagctgctttttgcctgtactgggtctctctggttagaccagatctgagcctgggagctctctggctaactagggaacccactgcttaagcctcaataaagcttgccttgagtgcttcaagtagtgtgtgcccgtctgttgtgtgactctggtaactagagatccctcagacccttttagtcagtgtggaaaatctctagcagtggcgcccgaacagggacttgaaagcgaaagggaaaccagaggagctctctcgacgcaggactcggcttgctgaagcgcgcacggcaagaggcgaggggcggcgactggtgagtacgccaaaaattttgactagcggaggctagaaggagagagatgggtgcgagagcgtcagtattaagcgggggagaattagatcgcgatgggaaaaaattcggttaaggccagggggaaagaaaaaatataaattaaaacatatagtatgggcaagcagggagctagaacgattcgcagttaatcctggcctgttagaaacatcagaaggctgtagacaaatactgggacagctacaaccatcccttcagacaggatcagaagaacttagatcattatataatacagtagcaaccctctattgtgtgcatcaaaggatagagataaaagacaccaaggaagctttagacaagatagaggaagagcaaaacaaaagtaagaccaccgcacagcaagcggccggccgctgatcttcagacctggaggaggagatatgagggacaattggagaagtgaattatataaatataaagtagtaaaaattgaaccattaggagtagcacccaccaaggcaaagagaagagtggtgcagagagaaaaaagagcagtgggaataggagctttgttccttgggttcttgggagcagcaggaagcactatgggcgcagcgtcaatgacgctgacggtacaggccagacaattattgtctggtatagtgcagcagcagaacaatttgctgagggctattgaggcgcaacagcatctgttgcaactcacagtctggggcatcaagcagctccaggcaagaatcctggctgtggaaagatacctaaaggatcaacagctcctggggatttggggttgctctggaaaactcatttgcaccactgctgtgccttggaatgctagttggagtaataaatctctggaacagatttggaatcacacgacctggatggagtgggacagagaaattaacaattacacaagcttaatacactccttaattgaagaatcgcaaaaccagcaagaaaagaatgaacaagaattattggaattagataaatgggcaagtttgtggaattggtttaacataacaaattggctgtggtatataaaattattcataatgatagtaggaggcttggtaggtttaagaatagtttttgctgtactttctatagtgaatagagttaggcagggatattcaccattatcgtttcagacccacctcccaaccccgaggggacccgacaggcccgaaggaatagaagaagaaggtggagagagagacagagacagatccattcgattagtgaacggatctcgacggtatcgcctttaaaagaaaaggggggattggggggtacagtgcaggggaaagaatagtagacataatagcaacagacatacaaactaaagaattacaaaaacaaattacaaaaattcaaaattttcgggtttattacagggacagcagagatccagtttatcgatctgcagagggccctgcgtatgagtgcaagtgggttttaggaccaggatgaggcggggtgggggtgcctacctgacgaccgaccccgacccactggacaagcacccaacccccattccccaaattgcgcatcccctatcagagagggggaggggaaacaggatgcggcgaggcgcgtgcgcactgccagcttcagcaccgcggacagtgccttcgcccccgcctggcggcgcgcgccaccgccgcctcagcactgaaggcgcgctgacgtcactcgccggtcccccgcaaactccccttcccggccaccttggtcgcgtccgcgccgccgccggcccagccggaccgcaccacgcgaggcgcgagataggggggcacgggcgcgaccatctgcgctgcggcgccggcgactcagcgctgcctcagtctgcggtgggcagcggaggagtcgtgtcgtgcctgagagcgcagggatctatttccggtgaattcgccaccatggcagagccccggcaggagttcgaggttatggaggatcacgccgggacctatggattgggcgataggaaagatcagggcgggtatactatgcatcaggaccaggaaggcgacacggacgctggtctcaaggaaagcccacttcagacgccgacagaggacgggtctgaggaacctgggagtgaaacttctgacgctaagtctacgcctactgcggaggcggaggaggcaggaataggagacacaccatcacttgaagacgaggcagcaggacacgtaacccaagcgagaatggtttctaagtccaaagatggaaccggatccgatgacaaaaaggccaagggagcagatggcaaaacaaaaataacgacaccgaggggtgcggctccccccggtcaaaagggacaggcaaatgccacgcgcatccctgctaaaacacccccggcgccgaaaacccccccttcatccggagagccacccaagtctggtgatagaagcgggtatagttcccccggtagtccggggactccaggatcacgcagcagaacgccatccctgccaaccccacccactagagagcccaaaaaggtcgcagtcgttcgcactccgccaaaaagcccttcctcagcgaaaagccgcctgcagacggcacctgtccccatgcctgaccttaaaaatgttaaaagcaaaatcggtagtaccgaaaatctcaagcatcagccaggaggggggaaggttcagatcatcaataagaagctggacctgtctaacgtgcagagcaagtgtggaagcaaagataacataaagcacgttttggggggcggaagcgtacagattgtgtataagccggtggacctctcaaaagtaacattcaagtgtgggagtctgggcaacatccatcacaaacccgggggcggtcaggtagaggtgaaaagcgaaaagctcgattttaaggatagggtacagagtaaaattgggtctctggacaacataacacacgtaccaggcggaggcaataagaagatagaaacgcataaactcacgttccgagagaacgctaaagcaaagactgaccacggggctgagattgtatacaagagtccggtcgtctctggggacacttccccccgacacctttctaacgttagttccactggtagtattgacatggtcgacagccctcaacttgccactttggcagacgaggtcagtgctagtcttgcaaagcagggcttggtgagcaagggcgaggagctgttcaccggggtggtgcccatcctggtcgagctggacggcgacgtaaacggccacaagttcagcgtgtccggcgagggcgagggcgatgccacctacggcaagctgaccctgaagttcatctgcaccaccggcaagctgcccgtgccctggcccaccctcgtgaccaccctgacctacggcgtgcagtgcttcagccgctaccccgaccacatgaagcagcacgacttcttcaagtccgccatgcccgaaggctacgtccaggagcgcaccatcttcttcaaggacgacggcaactacaagacccgcgccgaggtgaagttcgagggcgacaccctggtgaaccgcatcgagctgaagggcatcgacttcaaggaggacggcaacatcctggggcacaagctggagtacaactacaacagccacaacgtctatatcatggccgacaagcagaagaacggcatcaaggtgaacttcaagatccgccacaacatcgaggacggcagcgtgcagctcgccgaccactaccagcagaacacccccatcggcgacggccccgtgctgctgcccgacaaccactacctgagcacccagtccgccctgagcaaagaccccaacgagaagcgcgatcacatggtcctgctggagttcgtgaccgccgccgggatcactctcggcatggacgagctgtacaagtgaaattcgctcgagactagttctagagcggccgcggatcccgcccctctccctcccccccccctaacgttactggccgaagccgcttggaataaggccggtgtgcgtttgtctatatgttattttccaccatattgccgtcttttggcaatgtgagggcccggaaacctggccctgtcttcttgacgagcattcctaggggtctttcccctctcgccaaaggaatgcaaggtctgttgaatgtcgtgaaggaagcagttcctctggaagcttcttgaagacaaacaacgtctgtagcgaccctttgcaggcagcggaaccccccacctggcgacaggtgcctctgcggccaaaagccacgtgtataagatacacctgcaaaggcggcacaaccccagtgccacgttgtgagttggatagttgtggaaagagtcaaatggctctcctcaagcgtattcaacaaggggctgaaggatgcccagaaggtaccccattgtatgggatctgatctggggcctcggtgcacatgctttacatgtgtttagtcgaggttaaaaaaacgtctaggccccccgaaccacggggacgtggttttcctttgaaaaacacgatgataagcttgccacaacccgtaccaaagatggatagatccggaaagcctgaactcaccgcgacgtctgtcgagaagtttctgatcgaaaagttcgacagcgtctccgacctgatgcagctctcggagggcgaagaatctcgtgctttcagcttcgatgtaggagggcgtggatatgtcctgcgggtaaatagctgcgccgatggtttctacaaagatcgttatgtttatcggcactttgcatcggccgcgctcccgattccggaagtgcttgacattggggaattcagcgagagcctgacctattgcatctcccgccgtgcacagggtgtcacgttgcaagacctgcctgaaaccgaactgcccgctgttctgcagccggtcgcggaggccatggatgcgatcgctgcggccgatcttagccagacgagcgggttcggcccattcggaccgcaaggaatcggtcaatacactacatggcgtgatttcatatgcgcgattgctgatccccatgtgtatcactggcaaactgtgatggacgacaccgtcagtgcgtccgtcgcgcaggctctcgatgagctgatgctttgggccgaggactgccccgaagtccggcacctcgtgcacgcggatttcggctccaacaatgtcctgacggacaatggccgcataacagcggtcattgactggagcgaggcgatgttcggggattcccaatacgaggtcgccaacatcttcttctggaggccgtggttggcttgtatggagcagcagacgcgctacttcgagcggaggcatccggagcttgcaggatcgccgcggctccgggcgtatatgctccgcattggtcttgaccaactctatcagagcttggttgacggcaatttcgatgatgcagcttgggcgcagggtcgatgcgacgcaatcgtccgatccggagccgggactgtcgggcgtacacaaatcgcccgcagaagcgcggccgtctggaccgatggctgtgtagaagtactcgccgatagtggaaaccgacgccccagcactcgtccgagggcaaaggaatagacgcgtctggaacaatcaacctctggattacaaaatttgtgaaagattgactggtattcttaactatgttgctccttttacgctatgtggatacgctgctttaatgcctttgtatcatgctattgcttcccgtatggctttcattttctcctccttgtataaatcctggttgctgtctctttatgaggagttgtggcccgttgtcaggcaacgtggcgtggtgtgcactgtgtttgctgacgcaacccccactggttggggcattgccaccacctgtcagctcctttccgggactttcgctttccccctccctattgccacggcggaactcatcgccgcctgccttgcccgctgctggacaggggctcggctgttgggcactgacaattccgtggtgttgtcggggaagctgacgtcctttccatggctgctcgcctgtgttgccacctggattctgcgcgggacgtccttctgctacgtcccttcggccctcaatccagcggaccttccttcccgcggcctgctgccggctctgcggcctcttccgcgtcttcgccttcgccctcagacgagtcggatctccctttgggccgcctccccgcctggaattaattctgcagtcgagacctagaaaaacatggagcaatcacaagtagcaatacagcagctaccaatgctgattgtgcctggctagaagcacaagaggaggaggaggtgggttttccagtcacacctcaggtacctttaagaccaatgacttacaaggcagctgtagatcttagccactttttaaaagaaaagaggggactggaagggctaattcactcccaacgaagacaagatatccttgatctgtggatctaccacacacaaggctacttccctgattagcagaactacacaccagggccaggggtcagatatccactgacctttggatggtgctacaagctagtaccagttgagccagataaggtagaagaggccaataaaggagagaacaccagcttgttacaccctgtgagcctgcatgggatggatgacccggagagagaagtgttagagtggaggtttgacagccgcctagcatttcatcacgtggcccgagagctgcatccggagtacttcaagaactgctgatatcgagcttgctacaagggactttccgctggggactttccagggaggcgtggcctgggcgggactggggagtggcgagccctcagatcctgcatataagcagctgctttttgcctgtactgggtctctctggttagaccagatctgagcctgggagctctctggctaactagggaacccactgcttaagcctcaataaagcttgccttgagtgcttcaagtagtgtgtgcccgtctgttgtgtgactctggtaactagagatccctcagacccttttagtcagtgtggaaaatctctagcagtagtagttcatgtcatcttattattcagtatttataacttgcaaagaaatgaatatcagagagtgagaggccttgacattgctagcgtttaccgtcgacctctagctagagcttggcgtaatcatggtcatagctgtttcctgtgtgaaattgttatccgctcacaattccacacaacatacgagccggaagcataaagtgtaaagcctggggtgcctaatgagtgagctaactcacattaattgcgttgcgctcactgcccgctttccagtcgggaaacctgtcgtgccagctgcattaatgaatcggccaacgcgcggggagaggcggtttgcgtattgggcgctcttccgcttcctcgctcactgactcgctgcgctcggtcgttcggctgcggcgagcggtatcagctcactcaaaggcggtaatacggttatccacagaatcaggggataacgcaggaaagaacatgtgagcaaaaggccagcaaaaggccaggaaccgtaaaaaggccgcgttgctggcgtttttccataggctccgcccccctgacgagcatcacaaaaatcgacgctcaagtcagaggtggcgaaacccgacaggactataaagataccaggcgtttccccctggaagctccctcgtgcgctctcctgttccgaccctgccgcttaccggatacctgtccgcctttctcccttcgggaagcgtggcgctttctcatagctcacgctgtaggtatctcagttcggtgtaggtcgttcgctccaagctgggctgtgtgcacgaaccccccgttcagcccgaccgctgcgccttatccggtaactatcgtcttgagtccaacccggtaagacacgacttatcgccactggcagcagccactggtaacaggattagcagagcgaggtatgtaggcggtgctacagagttcttgaagtggtggcctaactacggctacactagaagaacagtatttggtatctgcgctctgctgaagccagttaccttcggaaaaagagttggtagctcttgatccggcaaacaaaccaccgctggtagcggtggtttttttgtttgcaagcagcagattacgcgcagaaaaaaaggatctcaagaagatcctttgatcttttctacggggtctgacgctcagtggaacgaaaactcacgttaagggattttggtcatgagattatcaaaaaggatcttcacctagatccttttaaattaaaaatgaagttttaaatcaatctaaagtatatatgagtaaacttggtctgacagttaccaatgcttaatcagtgaggcacctatctcagcgatctgtctatttcgttcatccatagttgcctgactccccgtcgtgtagataactacgatacgggagggcttaccatctggccccagtgctgcaatgataccgcgagacccacgctcaccggctccagatttatcagcaataaaccagccagccggaagggccgagcgcagaagtggtcctgcaactttatccgcctccatccagtctattaattgttgccgggaagctagagtaagtagttcgccagttaatagtttgcgcaacgttgttgccattgctacaggcatcgtggtgtcacgctcgtcgtttggtatggcttcattcagctccggttcccaacgatcaaggcgagttacatgatcccccatgttgtgcaaaaaagcggttagctccttcggtcctccgatcgttgtcagaagtaagttggccgcagtgttatcactcatggttatggcagcactgcataattctcttactgtcatgccatccgtaagatgcttttctgtgactggtgagtactcaaccaagtcattctgagaatagtgtatgcggcgaccgagttgctcttgcccggcgtcaatacgggataataccgcgccacatagcagaactttaaaagtgctcatcattggaaaacgttcttcggggcgaaaactctcaaggatcttaccgctgttgagatccagttcgatgtaacccactcgtgcacccaactgatcttcagcatcttttactttcaccagcgtttctgggtgagcaaaaacaggaaggcaaaatgccgcaaaaaagggaataagggcgacacggaaatgttgaatactcatactcttcctttttcaatattattgaagcatttatcagggttattgtctcatgagcggatacatatttgaatgtatttagaaaaataaacaaataggggttccgcgcacatttccccgaaaagtgccacctgacgtcgacggatcgggagatcaacttgtttattgcagcttataatggttacaaataaagcaatagcatcacaaatttcacaaataaagcatttttttcactgcattctagttgtggtttgtccaaactcatcaatgtatcttatcatgtctggatcaactggataactcaagctaaccaaaatcatcccaaacttcccaccccataccctattaccactgccaattacctgtggtttcatttactctaaacctgtgattcctctgaattattttcattttaaagaaattgtatttgttaaatatgtactacaaacttagtagt

SEQ ID NO: 80 - DNA, 10350 bp, Artificial Sequence
  Synthetic
  misc_feature (1)..(635): LTR
  misc_feature (636)..(653): PBS
  misc_feature (685)..(822): Packaging\signal
  misc_feature (1303)..(1536): RRE
  misc_feature (2028)..(2151): cPPT
  misc_feature (2185)..(2668): hSynapsin promoter
  misc_feature (2681)..(3397): eGFP
  misc_feature (3398)..(4633): CoHu hTau-412 (1NR4) 3MUT
  misc_feature (4640)..(4671): MCS
  misc_feature (4672)..(5270): IRES
  misc_feature (5271)..(6305): HygR
  misc_feature (6319)..(6910): WPRE
  misc_feature (7113)..(7749): LTR
  misc_feature (8218)..(8891): pUC\origin
  misc_feature (9036)..(10032): AmpR
tggaagggctaattcactcccaaagaagacaagatatccttgatctgtggatctaccacacacaaggctacttccctgattagcagaactacacaccagggccaggggtcagatatccactgacctttggatggtgctacaagctagtaccagttgagccagataaggtagaagaggccaataaaggagagaacaccagcttgttacaccctgtgagcctgcatgggatggatgacccggagagagaagtgttagagtggaggtttgacagccgcctagcatttcatcacgtggcccgagagctgcatccggagtacttcaagaactgctgatatcgagcttgctacaagggactttccgctggggactttccagggaggcgtggcctgggcgggactggggagtggcgagccctcagatcctgcatataagcagctgctttttgcctgtactgggtctctctggttagaccagatctgagcctgggagctctctggctaactagggaacccactgcttaagcctcaataaagcttgccttgagtgcttcaagtagtgtgtgcccgtctgttgtgtgactctggtaactagagatccctcagacccttttagtcagtgtggaaaatctctagcagtggcgcccgaacagggacttgaaagcgaaagggaaaccagaggagctctctcgacgcaggactcggcttgctgaagcgcgcacggcaagaggcgaggggcggcgactggtgagtacgccaaaaattttgactagcggaggctagaaggagagagatgggtgcgagagcgtcagtattaagcgggggagaattagatcgcgatgggaaaaaattcggttaaggccagggggaaagaaaaaatataaattaaaacatatagtatgggcaagcagggagctagaacgattcgcagttaatcctggcctgttagaaacatcagaaggctgtagacaaatactgggacagctacaaccatcccttcagacaggatcagaagaacttagatcattatataatacagtagcaaccctctattgtgtgcatcaaaggatagagataaaagacaccaaggaagctttagacaagatagaggaagagcaaaacaaaagtaagaccaccgcacagcaagcggccggccgctgatcttcagacctggaggaggagatatgagggacaattggagaagtgaattatataaatataaagtagtaaaaattgaaccattaggagtagcacccaccaaggcaaagagaagagtggtgcagagagaaaaaagagcagtgggaataggagctttgttccttgggttcttgggagcagcaggaagcactatgggcgcagcgtcaatgacgctgacggtacaggccagacaattattgtctggtatagtgcagcagcagaacaatttgctgagggctattgaggcgcaacagcatctgttgcaactcacagtctggggcatcaagcagctccaggcaagaatcctggctgtggaaagatacctaaaggatcaacagctcctggggatttggggttgctctggaaaactcatttgcaccactgctgtgccttggaatgctagttggagtaataaatctctggaacagatttggaatcacacgacctggatggagtgggacagagaaattaacaattacacaagcttaatacactccttaattgaagaatcgcaaaaccagcaagaaaagaatgaacaagaattattggaattagataaatgggcaagtttgtggaattggtttaacataacaaattggctgtggtatataaaattattcataatgatagtaggaggcttggtaggtttaagaatagtttttgctgtactttctatagtgaatagagttaggcagggatattcaccattatcgtttcagacccacctcccaaccccgaggggacccgacaggcccgaaggaatagaagaagaaggtggagagagagacagagacagatccattcgattagtgaacggatctcgacggtatcgcctttaaaagaaaaggggggattggggggtacagtgcaggggaaagaatagtagacataatagcaacagacatacaaactaaagaattacaaaaacaaattacaaaaattcaaaattttcgggtttattacagggacagcagagatccagtttatcgatctgcagagggccctgcgtatgagtgcaagtgggttttaggaccaggatgaggcggggtgggggtgcctacctgacgaccgaccccgacccactggacaagcacccaacccccattccccaaattgcgcatcccctatcagagagggggaggggaaacaggatgcggcgaggcgcgtgcgcactgccagcttcagcaccgcggacagtgccttcgcccccgcctggcggcgcgcgccaccgccgcctcagcactgaaggcgcgctgacgtcactcgccggtcccccgcaaactccccttcccggccaccttggtcgcgtccgcgccgccgccggcccagccggaccgcaccacgcgaggcgcgagataggggggcacgggcgcgaccatctgcgctgcggcgccggcgactcagcgctgcctcagtctgcggtgggcagcggaggagtcgtgtcgtgcctgagagcgcagggatctatttccggtgaattcgccaccatggtgagcaagggcgaggagctgttcaccggggtggtgcccatcctggtcgagctggacggcgacgtaaacggccacaagttcagcgtgtccggcgagggcgagggcgatgccacctacggcaagctgaccctgaagttcatctgcaccaccggcaagctgcccgtgccctggcccaccctcgtgaccaccctgacctacggcgtgcagtgcttcagccgctaccccgaccacatgaagcagcacgacttcttcaagtccgccatgcccgaaggctacgtccaggagcgcaccatcttcttcaaggacgacggcaactacaagacccgcgccgaggtgaagttcgagggcgacaccctggtgaaccgcatcgagctgaagggcatcgacttcaaggaggacggcaacatcctggggcacaagctggagtacaactacaacagccacaacgtctatatcatggccgacaagcagaagaacggcatcaaggtgaacttcaagatccgccacaacatcgaggacggcagcgtgcagctcgccgaccactaccagcagaacacccccatcggcgacggccccgtgctgctgcccgacaaccactacctgagcacccagtccgccctgagcaaagaccccaacgagaagcgcgatcacatggtcctgctggagttcgtgaccgccgccgggatcactctcggcatggacgagctgtacaaggcagagccccggcaggagttcgaggttatggaggatcacgccgggacctatggattgggcgataggaaagatcagggcgggtatactatgcatcaggaccaggaaggcgacacggacgctggtctcaaggaaagcccacttcagacgccgacagaggacgggtctgaggaacctgggagtgaaacttctgacgctaagtctacgcctactgcggaggcggaggaggcaggaataggagacacaccatcacttgaagacgaggcagcaggacacgtaacccaagcgagaatggtttctaagtccaaagatggaaccggatccgatgacaaaaaggccaagggagcagatggcaaaacaaaaataacgacaccgaggggtgcggctccccccggtcaaaagggacaggcaaatgccacgcgcatccctgctaaaacacccccggcgccgaaaacccccccttcatccggagagccacccaagtctggtgatagaagcgggtatagttcccccggtagtccggggactccaggatcacgcagcagaacgccatccctgccaaccccacccactagagagcccaaaaaggtcgcagtcgttcgcactccgccaaaaagcccttcctcagcgaaaagccgcctgcagacggcacctgtccccatgcctgaccttaaaaatgttaaaagcaaaatcggtagtaccgaaaatctcaagcatcagccaggaggggggaaggttcagatcatcaataagaagctggacctgtctaacgtgcagagcaagtgtggaagcaaagataacataaagcacgttttggggggcggaagcgtacagattgtgtataagccggtggacctctcaaaagtaacattcaagtgtgggagtctgggcaacatccatcacaaacccgggggcggtcaggtagaggtgaaaagcgaaaagctcgattttaaggatagggtacagagtaaaattgggtctctggacaacataacacacgtaccaggcggaggcaataagaagatagaaacgcataaactcacgttccgagagaacgctaaagcaaagactgaccacggggctgagattgtatacaagagtccggtcgtctctggggacacttccccccgacacctttctaacgttagttccactggtagtattgacatggtcgacagccctcaacttgccactttggcagacgaggtcagtgctagtcttgcaaagcagggcttgtgaaattcgctcgagactagttctagagcggccgcggatcccgcccctctccctcccccccccctaacgttactggccgaagccgcttggaataaggccggtgtgcgtttgtctatatgttattttccaccatattgccgtcttttggcaatgtgagggcccggaaacctggccctgtcttcttgacgagcattcctaggggtctttcccctctcgccaaaggaatgcaaggtctgttgaatgtcgtgaaggaagcagttcctctggaagcttcttgaagacaaacaacgtctgtagcgaccctttgcaggcagcggaaccccccacctggcgacaggtgcctctgcggccaaaagccacgtgtataagatacacctgcaaaggcggcacaaccccagtgccacgttgtgagttggatagttgtggaaagagtcaaatggctctcctcaagcgtattcaacaaggggctgaaggatgcccagaaggtaccccattgtatgggatctgatctggggcctcggtgcacatgctttacatgtgtttagtcgaggttaaaaaaacgtctaggccccccgaaccacggggacgtggttttcctttgaaaaacacgatgataagcttgccacaacccgtaccaaagatggatagatccggaaagcctgaactcaccgcgacgtctgtcgagaagtttctgatcgaaaagttcgacagcgtctccgacctgatgcagctctcggagggcgaagaatctcgtgctttcagcttcgatgtaggagggcgtggatatgtcctgcgggtaaatagctgcgccgatggtttctacaaagatcgttatgtttatcggcactttgcatcggccgcgctcccgattccggaagtgcttgacattggggaattcagcgagagcctgacctattgcatctcccgccgtgcacagggtgtcacgttgcaagacctgcctgaaaccgaactgcccgctgttctgcagccggtcgcggaggccatggatgcgatcgctgcggccgatcttagccagacgagcgggttcggcccattcggaccgcaaggaatcggtcaatacactacatggcgtgatttcatatgcgcgattgctgatccccatgtgtatcactggcaaactgtgatggacgacaccgtcagtgcgtccgtcgcgcaggctctcgatgagctgatgctttgggccgaggactgccccgaagtccggcacctcgtgcacgcggatttcggctccaacaatgtcctgacggacaatggccgcataacagcggtcattgactggagcgaggcgatgttcggggattcccaatacgaggtcgccaacatcttcttctggaggccgtggttggcttgtatggagcagcagacgcgctacttcgagcggaggcatccggagcttgcaggatcgccgcggctccgggcgtatatgctccgcattggtcttgaccaactctatcagagcttggttgacggcaatttcgatgatgcagcttgggcgcagggtcgatgcgacgcaatcgtccgatccggagccgggactgtcgggcgtacacaaatcgcccgcagaagcgcggccgtctggaccgatggctgtgtagaagtactcgccgatagtggaaaccgacgccccagcactcgtccgagggcaaaggaatagacgcgtctggaacaatcaacctctggattacaaaatttgtgaaagattgactggtattcttaactatgttgctccttttacgctatgtggatacgctgctttaatgcctttgtatcatgctattgcttcccgtatggctttcattttctcctccttgtataaatcctggttgctgtctctttatgaggagttgtggcccgttgtcaggcaacgtggcgtggtgtgcactgtgtttgctgacgcaacccccactggttggggcattgccaccacctgtcagctcctttccgggactttcgctttccccctccctattgccacggcggaactcatcgccgcctgccttgcccgctgctggacaggggctcggctgttgggcactgacaattccgtggtgttgtcggggaagctgacgtcctttccatggctgctcgcctgtgttgccacctggattctgcgcgggacgtccttctgctacgtcccttcggccctcaatccagcggaccttccttcccgcggcctgctgccggctctgcggcctcttccgcgtcttcgccttcgccctcagacgagtcggatctccctttgggccgcctccccgcctggaattaattctgcagtcgagacctagaaaaacatggagcaatcacaagtagcaatacagcagctaccaatgctgattgtgcctggctagaagcacaagaggaggaggaggtgggttttccagtcacacctcaggtacctttaagaccaatgacttacaaggcagctgtagatcttagccactttttaaaagaaaagaggggactggaagggctaattcactcccaacgaagacaagatatccttgatctgtggatctaccacacacaaggctacttccctgattagcagaactacacaccagggccaggggtcagatatccactgacctttggatggtgctacaagctagtaccagttgagccagataaggtagaagaggccaataaaggagagaacaccagcttgttacaccctgtgagcctgcatgggatggatgacccggagagagaagtgttagagtggaggtttgacagccgcctagcatttcatcacgtggcccgagagctgcatccggagtacttcaagaactgctgatatcgagcttgctacaagggactttccgctggggactttccagggaggcgtggcctgggcgggactggggagtggcgagccctcagatcctgcatataagcagctgctttttgcctgtactgggtctctctggttagaccagatctgagcctgggagctctctggctaactagggaacccactgcttaagcctcaataaagcttgccttgagtgcttcaagtagtgtgtgcccgtctgttgtgtgactctggtaactagagatccctcagacccttttagtcagtgtggaaaatctctagcagtagtagttcatgtcatcttattattcagtatttataacttgcaaagaaatgaatatcagagagtgagaggccttgacattgctagcgtttaccgtcgacctctagctagagcttggcgtaatcatggtcatagctgtttcctgtgtgaaattgttatccgctcacaattccacacaacatacgagccggaagcataaagtgtaaagcctggggtgcctaatgagtgagctaactcacattaattgcgttgcgctcactgcccgctttccagtcgggaaacctgtcgtgccagctgcattaatgaatcggccaacgcgcggggagaggcggtttgcgtattgggcgctcttccgcttcctcgctcactgactcgctgcgctcggtcgttcggctgcggcgagcggtatcagctcactcaaaggcggtaatacggttatccacagaatcaggggataacgcaggaaagaacatgtgagcaaaaggccagcaaaaggccaggaaccgtaaaaaggccgcgttgctggcgtttttccataggctccgcccccctgacgagcatcacaaaaatcgacgctcaagtcagaggtggcgaaacccgacaggactataaagataccaggcgtttccccctggaagctccctcgtgcgctctcctgttccgaccctgccgcttaccggatacctgtccgcctttctcccttcgggaagcgtggcgctttctcatagctcacgctgtaggtatctcagttcggtgtaggtcgttcgctccaagctgggctgtgtgcacgaaccccccgttcagcccgaccgctgcgccttatccggtaactatcgtcttgagtccaacccggtaagacacgacttatcgccactggcagcagccactggtaacaggattagcagagcgaggtatgtaggcggtgctacagagttcttgaagtggtggcctaactacggctacactagaagaacagtatttggtatctgcgctctgctgaagccagttaccttcggaaaaagagttggtagctcttgatccggcaaacaaaccaccgctggtagcggtggtttttttgtttgcaagcagcagattacgcgcagaaaaaaaggatctcaagaagatcctttgatcttttctacggggtctgacgctcagtggaacgaaaactcacgttaagggattttggtcatgagattatcaaaaaggatcttcacctagatccttttaaattaaaaatgaagttttaaatcaatctaaagtatatatgagtaaacttggtctgacagttaccaatgcttaatcagtgaggcacctatctcagcgatctgtctatttcgttcatccatagttgcctgactccccgtcgtgtagataactacgatacgggagggcttaccatctggccccagtgctgcaatgataccgcgagacccacgctcaccggctccagatttatcagcaataaaccagccagccggaagggccgagcgcagaagtggtcctgcaactttatccgcctccatccagtctattaattgttgccgggaagctagagtaagtagttcgccagttaatagtttgcgcaacgttgttgccattgctacaggcatcgtggtgtcacgctcgtcgtttggtatggcttcattcagctccggttcccaacgatcaaggcgagttacatgatcccccatgttgtgcaaaaaagcggttagctccttcggtcctccgatcgttgtcagaagtaagttggccgcagtgttatcactcatggttatggcagcactgcataattctcttactgtcatgccatccgtaagatgcttttctgtgactggtgagtactcaaccaagtcattctgagaatagtgtatgcggcgaccgagttgctcttgcccggcgtcaatacgggataataccgcgccacatagcagaactttaaaagtgctcatcattggaaaacgttcttcggggcgaaaactctcaaggatcttaccgctgttgagatccagttcgatgtaacccactcgtgcacccaactgatcttcagcatcttttactttcaccagcgtttctgggtgagcaaaaacaggaaggcaaaatgccgcaaaaaagggaataagggcgacacggaaatgttgaatactcatactcttcctttttcaatattattgaagcatttatcagggttattgtctcatgagcggatacatatttgaatgtatttagaaaaataaacaaataggggttccgcgcacatttccccgaaaagtgccacctgacgtcgacggatcgggagatcaacttgtttattgcagcttataatggttacaaataaagcaatagcatcacaaatttcacaaataaagcatttttttcactgcattctagttgtggtttgtccaaactcatcaatgtatcttatcatgtctggatcaactggataactcaagctaaccaaaatcatcccaaacttcccaccccataccctattaccactgccaattacctgtggtttcatttactctaaacctgtgattcctctgaattattttcattttaaagaaattgtatttgttaaatatgtactacaaacttagtagt

SEQ ID NO: 81 - DNA, 1236 bp, Artificial Sequence
  Synthetic
gctgagccccgacaggagttcgaggtaatggaggatcacgcagggacgtatggtctgggagacaggaaggatcaaggcggctatacgatgcaccaggatcaggagggcgataccgatgcgggcctcaaagagtccccgcttcaaacaccaactgaggatgggagtgaggagccaggaagtgagacaagcgacgcgaaatcaacccctactgccgaagcggaggaggccgggatcggagatacaccatctctcgaagacgaagctgctggccacgtgacgcaagcacgaatggtgtccaaaagcaaagacggtacaggttctgacgacaaaaaggcgaagggggcagatgggaaaactaaaatcgccacgccccggggtgcggcgccgcctgggcagaaagggcaagcaaatgcgacgcgaatacctgccaagacgcctccggctcctaagaccccaccatcatctggtgaaccgcctaaaagcggggatcgaagcggttattcatcaccgggtagtccgggtacgccaggctctaggagcagaactccttcactgcccacgccccccacgcgcgaacctaagaaagtggcagtggtgcgaacacccccaaaaagcccctcaagtgcaaaatcacggctccagactgcacccgtaccgatgcccgatctcaaaaacgtgaaatctaagataggtagtacagagaatctgaagcatcaaccgggaggtggaaaggtgcagattatcaataagaaacttgacctgagtaacgttcaatccaagtgtggatcaaaagataatatcaagcacgtccctggaggcggttcagtgcagatcgtttacaaacctgttgatcttagcaaggtgacttccaagtgcgggtctctgggcaacattcatcacaaacctggtggagggcaagttgaggtcaaaagcgaaaagctcgacttcaaagatcgagttcagagcaagataggcagccttgataatattacccatgtccccggcggagggaacaagaagattgagactcataagttgacgttcagagaaaatgctaaagcgaaaacggatcatggcgcagaaatagtttataaatctcctgtggtcagtggtgacacttcacccaggcacctctcaaacgtgtcatcaacgggctcaatcgacatggtggattctccccaactcgcaacacttgctgatgaggtaagtgccagcctcgcaaagcaaggactctaa

SEQ ID NO: 82 - protein, 411 aa, Artificial Sequence
  Synthetic
AEPRQEFEVMEDHAGTYGLGDRKDQGGYTMHQDQEGDTDAGLKESPLQTPTEDGSEEPGSETSDAKSTPTAEAEEAGIGDTPSLEDEAAGHVTQARMVSKSKDGTGSDDKKAKGADGKTKIATPRGAAPPGQKGQANATRIPAKTPPAPKTPPSSGEPPKSGDRSGYSSPGSPGTPGSRSRTPSLPTPPTREPKKVAVVRTPPKSPSSAKSRLQTAPVPMPDLKNVKSKIGSTENLKHQPGGGKVQIINKKLDLSNVQSKCGSKDNIKHVPGGGSVQIVYKPVDLSKVTSKCGSLGNIHHKPGGGQVEVKSEKLDFKDRVQSKIGSLDNITHVPGGGNKKIETHKLTFRENAKAKTDHGAEIVYKSPVVSGDTSPRHLSNVSSTGSIDMVDSPQLATLADEVSASLAKQGL

SEQ ID NO: 83 - DNA, 1236 bp, Artificial Sequence
  Synthetic
gcagagccccggcaggagttcgaggttatggaggatcacgccgggacctatggattgggcgataggaaagatcagggcgggtatactatgcatcaggaccaggaaggcgacacggacgctggtctcaaggaaagcccacttcagacgccgacagaggacgggtctgaggaacctgggagtgaaacttctgacgctaagtctacgcctactgcggaggcggaggaggcaggaataggagacacaccatcacttgaagacgaggcagcaggacacgtaacccaagcgagaatggtttctaagtccaaagatggaaccggatccgatgacaaaaaggccaagggagcagatggcaaaacaaaaataacgacaccgaggggtgcggctccccccggtcaaaagggacaggcaaatgccacgcgcatccctgctaaaacacccccggcgccgaaaacccccccttcatccggagagccacccaagtctggtgatagaagcgggtatagttcccccggtagtccggggactccaggatcacgcagcagaacgccatccctgccaaccccacccactagagagcccaaaaaggtcgcagtcgttcgcactccgccaaaaagcccttcctcagcgaaaagccgcctgcagacggcacctgtccccatgcctgaccttaaaaatgttaaaagcaaaatcggtagtaccgaaaatctcaagcatcagccaggaggggggaaggttcagatcatcaataagaagctggacctgtctaacgtgcagagcaagtgtggaagcaaagataacataaagcacgttttggggggcggaagcgtacagattgtgtataagccggtggacctctcaaaagtaacattcaagtgtgggagtctgggcaacatccatcacaaacccgggggcggtcaggtagaggtgaaaagcgaaaagctcgattttaaggatagggtacagagtaaaattgggtctctggacaacataacacacgtaccaggcggaggcaataagaagatagaaacgcataaactcacgttccgagagaacgctaaagcaaagactgaccacggggctgagattgtatacaagagtccggtcgtctctggggacacttccccccgacacctttctaacgttagttccactggtagtattgacatggtcgacagccctcaacttgccactttggcagacgaggtcagtgctagtcttgcaaagcagggcttgtga

SEQ ID NO: 84 - protein, 411 aa, Artificial Sequence
  Synthetic
AEPRQEFEVMEDHAGTYGLGDRKDQGGYTMHQDQEGDTDAGLKESPLQTPTEDGSEEPGSETSDAKSTPTAEAEEAGIGDTPSLEDEAAGHVTQARMVSKSKDGTGSDDKKAKGADGKTKITTPRGAAPPGQKGQANATRIPAKTPPAPKTPPSSGEPPKSGDRSGYSSPGSPGTPGSRSRTPSLPTPPTREPKKVAVVRTPPKSPSSAKSRLQTAPVPMPDLKNVKSKIGSTENLKHQPGGGKVQIINKKLDLSNVQSKCGSKDNIKHVLGGGSVQIVYKPVDLSKVTFKCGSLGNIHHKPGGGQVEVKSEKLDFKDRVQSKIGSLDNITHVPGGGNKKIETHKLTFRENAKAKTDHGAEIVYKSPVVSGDTSPRHLSNVSSTGSIDMVDSPQLATLADEVSASLAKQGL

SEQ ID NO: 85 - DNA, 14873 bp, Artificial Sequence
  Synthetic
  misc_feature (217)..(397): LTR
  misc_feature (444)..(569): HIV-1 Psi
  misc_feature (1062)..(1295): RRE
  misc_feature (1822)..(1939): cPPT/CTS
  misc_feature (4120)..(4195): gRNA Scaffold
  misc_feature (4487)..(4496): Kozak
  misc_feature (4493)..(8596): Cas9 CDS
  misc_feature (8597)..(8644): NLS
  misc_feature (8645)..(8668): FLAG
  misc_feature (8678)..(8734): P2A
  misc_feature (8735)..(9331): PuroR
  misc_feature (9347)..(9935): WPRE
  misc_feature (9818)..(9829): Factor Xa site
  misc_feature (10007)..(10240): LTR
  misc_feature (10542)..(10970): F1 ori
  misc_feature (11164)..(11299): SV40 ori
  misc_feature (11427)..(11801): BleoR
  misc_feature (12125)..(12141): Lac operator
  misc_feature (12194)..(12215): CAP binding site
  misc_feature (12503)..(13091): Ori
  misc_feature (13262)..(14122): AmpR
tgatgcggttttggcagtacatcaatgggcgtggatagcggtttgactcacggggatttccaagtctccaccccattgacgtcaatgggagtttgttttggcaccaaaatcaacgggactttccaaaatgtcgtaacaactccgccccattgacgcaaatgggcggtaggcgtgtacggtgggaggtctatataagcagcgcgttttgcctgtactgggtctctctggttagaccagatctgagcctgggagctctctggctaactagggaacccactgcttaagcctcaataaagcttgccttgagtgcttcaagtagtgtgtgcccgtctgttgtgtgactctggtaactagagatccctcagacccttttagtcagtgtggaaaatctctagcagtggcgcccgaacagggacttgaaagcgaaagggaaaccagaggagctctctcgacgcaggactcggcttgctgaagcgcgcacggcaagaggcgaggggcggcgactggtgagtacgccaaaaattttgactagcggaggctagaaggagagagatgggtgcgagagcgtcagtattaagcgggggagaattagatcgcgatgggaaaaaattcggttaaggccagggggaaagaaaaaatataaattaaaacatatagtatgggcaagcagggagctagaacgattcgcagttaatcctggcctgttagaaacatcagaaggctgtagacaaatactgggacagctacaaccatcccttcagacaggatcagaagaacttagatcattatataatacagtagcaaccctctattgtgtgcatcaaaggatagagataaaagacaccaaggaagctttagacaagatagaggaagagcaaaacaaaagtaagaccaccgcacagcaagcggccgctgatcttcagacctggaggaggagatatgagggacaattggagaagtgaattatataaatataaagtagtaaaaattgaaccattaggagtagcacccaccaaggcaaagagaagagtggtgcagagagaaaaaagagcagtgggaataggagctttgttccttgggttcttgggagcagcaggaagcactatgggcgcagcgtcaatgacgctgacggtacaggccagacaattattgtctggtatagtgcagcagcagaacaatttgctgagggctattgaggcgcaacagcatctgttgcaactcacagtctggggcatcaagcagctccaggcaagaatcctggctgtggaaagatacctaaaggatcaacagctcctggggatttggggttgctctggaaaactcatttgcaccactgctgtgccttggaatgctagttggagtaataaatctctggaacagatttggaatcacacgacctggatggagtgggacagagaaattaacaattacacaagcttaatacactccttaattgaagaatcgcaaaaccagcaagaaaagaatgaacaagaattattggaattagataaatgggcaagtttgtggaattggtttaacataacaaattggctgtggtatataaaattattcataatgatagtaggaggcttggtaggtttaagaatagtttttgctgtactttctatagtgaatagagttaggcagggatattcaccattatcgtttcagacccacctcccaaccccgaggggacccgacaggcccgaaggaatagaagaagaaggtggagagagagacagagacagatccattcgattagtgaacggatcggcactgcgtgcgccaattctgcagacaaatggcagtattcatccacaattttaaaagaaaaggggggattggggggtacagtgcaggggaaagaatagtagacataatagcaacagacatacaaactaaagaattacaaaaacaaattacaaaaattcaaaattttcgggtttattacagggacagcagagatccagtttggttaattaaggtaccgagggcctatttcccatgattccttcatatttgcatatacgatacaaggctgttagagagataattagaattaatttgactgtaaacacaaagatattagtacaaaatacgtgacgtagaaagtaataatttcttgggtagtttgcagttttaaaattatgttttaaaatggactatcatatgcttaccgtaacttgaaagtatttcgatttcttggctttatatatcttgtggaaaggacgaaacaccggagacggttgtaaatgagcacacaaaatacacatgctaaaatattatattctatgacctttataaaatcaaccaaaatcttctttttaataactttagtatcaataattagaatttttatgttcctttttgcaaacttttaataaaaatgagcaaaataaaaaaacgctagttttagtaactcgcgttgttttcttcacctttaataatagctactccaccacttgttcctaagcggtcagctcctgcttcaatcattttttgagcatcttcaaatgttctaactccaccagctgctttaactaaagcattgtctttaacaactgacttcattagtttaacatcttcaaatgttgcacctgattttgaaaatcctgttgatgttttaacaaattctaatccagcttcaacagctatttcacaagctttcatgatttcttcttttgttaataaacaattttccataatacatttaacaacatgtgatccagctgctttttttacagctttcatgtcttctaaaactaattcataatttttgtcttttaatgcaccaatatttaataccatatcaatttctgttgcaccatctttaattgcttcagaaacttcgaatgcttttgtagctgttgtgcatgcacctagaggaaaacctacaacatttgttattcctacatttgtgccttttaataattctttacaatagcttgttcaatatgaattaacacaaactgttgcaaaatcaaattcaattgcttcatcacataattgtttaatttcagctttcgtagcatcttgttttaataatgtgtgatctatatatttgtttagtttcattttttctcctatatattcatttttaattttaattctttaataatttcgtctactttaactttagcgttttgaacagattcaccaacacctataaaataaatttttagtttaggttcagttccacttgggcgaacagcaaatcatgacttatcttctaaataaaattttagtaagtcttgtcctggcatattatacattccatcgatgtagtcttcaacattaacaactttaagtccagcaatttgagttaagggtgttgctctcaatgatttcattaatggttcaatttttaatttcttttcttctggtttaaaattcaagtttaaagtgaaagtgtaatatgcacccatttctttaaataaatcttctaaatagtctactaatgttttattttgttttttataaaatcaagcagcctctgctattaatatagaagcttgtattccatctttatctctagctgagtcatcaattacatatccataactttcttcataagcaaaaacaaaatttaatccgttatcttcttctttagcaatttctctacccattcatttaaatccagttaaagtttttacaatattaactccatatttttcatgagcgattctatcacccaaatcacttgttacaaaacttgaatatagagccggattttttggaatgctatttaagcgttttagatttgataattttcaatcaattaaaattggtcctgtttgatttccatctaatcttacaaaatgaccatcatgttttattgccattccaaatctgtcagcatctgggtcattcataataataatatctgcatcatgtttaataccatattcaagcggtatttttcatgcaggatcaaattctggatttggatttacaacatttttaaatgtttcatcttcaaatgcatgctcttcaacctcaataacgttatatcctgattcacgtaatatttttggggtaaatttagttcctgttccattaactgcgctaaaaataatttttaaatcttttttagcttcttgctcttttttgtacgtctctgttttagagctagaaatagcaagttaaaataaggctagtccgttatcaacttgaaaaagtggcaccgagtcggtgcttttttgaattcgctagctaggtcttgaaaggagtgggaattggctccggtgcccgtcagtgggcagagcgcacatcgcccacagtccccgagaagttggggggaggggtcggcaattgatccggtgcctagagaaggtggcgcggggtaaactgggaaagtgatgtcgtgtactggctccgcctttttcccgagggtgggggagaaccgtatataagtgcagtagtcgccgtgaacgttctttttcgcaacgggtttgccgccagaacacaggaccggttctagagcgctgccaccatggacaagaagtacagcatcggcctggacatcggcaccaactctgtgggctgggccgtgatcaccgacgagtacaaggtgcccagcaagaaattcaaggtgctgggcaacaccgaccggcacagcatcaagaagaacctgatcggagccctgctgttcgacagcggcgaaacagccgaggccacccggctgaagagaaccgccagaagaagatacaccagacggaagaaccggatctgctatctgcaagagatcttcagcaacgagatggccaaggtggacgacagcttcttccacagactggaagagtccttcctggtggaagaggataagaagcacgagcggcaccccatcttcggcaacatcgtggacgaggtggcctaccacgagaagtaccccaccatctaccacctgagaaagaaactggtggacagcaccgacaaggccgacctgcggctgatctatctggccctggcccacatgatcaagttccggggccacttcctgatcgagggcgacctgaaccccgacaacagcgacgtggacaagctgttcatccagctggtgcagacctacaaccagctgttcgaggaaaaccccatcaacgccagcggcgtggacgccaaggccatcctgtctgccagactgagcaagagcagacggctggaaaatctgatcgcccagctgcccggcgagaagaagaatggcctgttcggaaacctgattgccctgagcctgggcctgacccccaacttcaagagcaacttcgacctggccgaggatgccaaactgcagctgagcaaggacacctacgacgacgacctggacaacctgctggcccagatcggcgaccagtacgccgacctgtttctggccgccaagaacctgtccgacgccatcctgctgagcgacatcctgagagtgaacaccgagatcaccaaggcccccctgagcgcctctatgatcaagagatacgacgagcaccaccaggacctgaccctgctgaaagctctcgtgcggcagcagctgcctgagaagtacaaagagattttcttcgaccagagcaagaacggctacgccggctacattgacggcggagccagccaggaagagttctacaagttcatcaagcccatcctggaaaagatggacggcaccgaggaactgctcgtgaagctgaacagagaggacctgctgcggaagcagcggaccttcgacaacggcagcatcccccaccagatccacctgggagagctgcacgccattctgcggcggcaggaagatttttacccattcctgaaggacaaccgggaaaagatcgagaagatcctgaccttccgcatcccctactacgtgggccctctggccaggggaaacagcagattcgcctggatgaccagaaagagcgaggaaaccatcaccccctggaacttcgaggaagtggtggacaagggcgcttccgcccagagcttcatcgagcggatgaccaacttcgataagaacctgcccaacgagaaggtgctgcccaagcacagcctgctgtacgagtacttcaccgtgtataacgagctgaccaaagtgaaatacgtgaccgagggaatgagaaagcccgccttcctgagcggcgagcagaaaaaggccatcgtggacctgctgttcaagaccaaccggaaagtgaccgtgaagcagctgaaagaggactacttcaagaaaatcgagtgcttcgactccgtggaaatctccggcgtggaagatcggttcaacgcctccctgggcacataccacgatctgctgaaaattatcaaggacaaggacttcctggacaatgaggaaaacgaggacattctggaagatatcgtgctgaccctgacactgtttgaggacagagagatgatcgaggaacggctgaaaacctatgcccacctgttcgacgacaaagtgatgaagcagctgaagcggcggagatacaccggctggggcaggctgagccggaagctgatcaacggcatccgggacaagcagtccggcaagacaatcctggatttcctgaagtccgacggcttcgccaacagaaacttcatgcagctgatccacgacgacagcctgacctttaaagaggacatccagaaagcccaggtgtccggccagggcgatagcctgcacgagcacattgccaatctggccggcagccccgccattaagaagggcatcctgcagacagtgaaggtggtggacgagctcgtgaaagtgatgggccggcacaagcccgagaacatcgtgatcgaaatggccagagagaaccagaccacccagaagggacagaagaacagccgcgagagaatgaagcggatcgaagagggcatcaaagagctgggcagccagatcctgaaagaacaccccgtggaaaacacccagctgcagaacgagaagctgtacctgtactacctgcagaatgggcgggatatgtacgtggaccaggaactggacatcaaccggctgtccgactacgatgtggaccatatcgtgcctcagagctttctgaaggacgactccatcgacaacaaggtgctgaccagaagcgacaagaaccggggcaagagcgacaacgtgccctccgaagaggtcgtgaagaagatgaagaactactggcggcagctgctgaacgccaagctgattacccagagaaagttcgacaatctgaccaaggccgagagaggcggcctgagcgaactggataaggccggcttcatcaagagacagctggtggaaacccggcagatcacaaagcacgtggcacagatcctggactcccggatgaacactaagtacgacgagaatgacaagctgatccgggaagtgaaagtgatcaccctgaagtccaagctggtgtccgatttccggaaggatttccagttttacaaagtgcgcgagatcaacaactaccaccacgcccacgacgcctacctgaacgccgtcgtgggaaccgccctgatcaaaaagtaccctaagctggaaagcgagttcgtgtacggcgactacaaggtgtacgacgtgcggaagatgatcgccaagagcgagcaggaaatcggcaaggctaccgccaagtacttcttctacagcaacatcatgaactttttcaagaccgagattaccctggccaacggcgagatccggaagcggcctctgatcgagacaaacggcgaaaccggggagatcgtgtgggataagggccgggattttgccaccgtgcggaaagtgctgagcatgccccaagtgaatatcgtgaaaaagaccgaggtgcagacaggcggcttcagcaaagagtctatcctgcccaagaggaacagcgataagctgatcgccagaaagaaggactgggaccctaagaagtacggcggcttcgacagccccaccgtggcctattctgtgctggtggtggccaaagtggaaaagggcaagtccaagaaactgaagagtgtgaaagagctgctggggatcaccatcatggaaagaagcagcttcgagaagaatcccatcgactttctggaagccaagggctacaaagaagtgaaaaaggacctgatcatcaagctgcctaagtactccctgttcgagctggaaaacggccggaagagaatgctggcctctgccggcgaactgcagaagggaaacgaactggccctgccctccaaatatgtgaacttcctgtacctggccagccactatgagaagctgaagggctcccccgaggataatgagcagaaacagctgtttgtggaacagcacaagcactacctggacgagatcatcgagcagatcagcgagttctccaagagagtgatcctggccgacgctaatctggacaaagtgctgtccgcctacaacaagcaccgggataagcccatcagagagcaggccgagaatatcatccacctgtttaccctgaccaatctgggagcccctgccgccttcaagtactttgacaccaccatcgaccggaagaggtacaccagcaccaaagaggtgctggacgccaccctgatccaccagagcatcaccggcctgtacgagacacggatcgacctgtctcagctgggaggcgacaagcgacctgccgccacaaagaaggctggacaggctaagaagaagaaagattacaaagacgatgacgataagggatccggcgcaacaaacttctctctgctgaaacaagccggagatgtcgaagagaatcctggaccgaccgagtacaagcccacggtgcgcctcgccacccgcgacgacgtccccagggccgtacgcaccctcgccgccgcgttcgccgactaccccgccacgcgccacaccgtcgatccggaccgccacatcgagcgggtcaccgagctgcaagaactcttcctcacgcgcgtcgggctcgacatcggcaaggtgtgggtcgcggacgacggcgccgcggtggcggtctggaccacgccggagagcgtcgaagcgggggcggtgttcgccgagatcggcccgcgcatggccgagttgagcggttcccggctggccgcgcagcaacagatggaaggcctcctggcgccgcaccggcccaaggagcccgcgtggttcctggccaccgtcggagtctcgcccgaccaccagggcaagggtctgggcagcgccgtcgtgctccccggagtggaggcggccgagcgcgccggggtgcccgccttcctggagacctccgcgccccgcaacctccccttctacgagcggctcggcttcaccgtcaccgccgacgtcgaggtgcccgaaggaccgcgcacctggtgcatgacccgcaagcccggtgcctgaacgcgttaagtcgacaatcaacctctggattacaaaatttgtgaaagattgactggtattcttaactatgttgctccttttacgctatgtggatacgctgctttaatgcctttgtatcatgctattgcttcccgtatggctttcattttctcctccttgtataaatcctggttgctgtctctttatgaggagttgtggcccgttgtcaggcaacgtggcgtggtgtgcactgtgtttgctgacgcaacccccactggttggggcattgccaccacctgtcagctcctttccgggactttcgctttccccctccctattgccacggcggaactcatcgccgcctgccttgcccgctgctggacaggggctcggctgttgggcactgacaattccgtggtgttgtcggggaaatcatcgtcctttccttggctgctcgcctgtgttgccacctggattctgcgcgggacgtccttctgctacgtcccttcggccctcaatccagcggaccttccttcccgcggcctgctgccggctctgcggcctcttccgcgtcttcgccttcgccctcagacgagtcggatctccctttgggccgcctccccgcgtcgactttaagaccaatgacttacaaggcagctgtagatcttagccactttttaaaagaaaaggggggactggaagggctaattcactcccaacgaagacaagatctgctttttgcttgtactgggtctctctggttagaccagatctgagcctgggagctctctggctaactagggaacccactgcttaagcctcaataaagcttgccttgagtgcttcaagtagtgtgtgcccgtctgttgtgtgactctggtaactagagatccctcagacccttttagtcagtgtggaaaatctctagcagggcccgtttaaacccgctgatcagcctcgactgtgccttctagttgccagccatctgttgtttgcccctcccccgtgccttccttgaccctggaaggtgccactcccactgtcctttcctaataaaatgaggaaattgcatcgcattgtctgagtaggtgtcattctattctggggggtggggtggggcaggacagcaagggggaggattgggaagacaatagcaggcatgctggggatgcggtgggctctatggcttctgaggcggaaagaaccagctggggctctagggggtatccccacgcgccctgtagcggcgcattaagcgcggcgggtgtggtggttacgcgcagcgtgaccgctacacttgccagcgccctagcgcccgctcctttcgctttcttcccttcctttctcgccacgttcgccggctttccccgtcaagctctaaatcgggggctccctttagggttccgatttagtgctttacggcacctcgaccccaaaaaacttgattagggtgatggttcacgtagtgggccatcgccctgatagacggtttttcgccctttgacgttggagtccacgttctttaatagtggactcttgttccaaactggaacaacactcaaccctatctcggtctattcttttgatttataagggattttgccgatttcggcctattggttaaaaaatgagctgatttaacaaaaatttaacgcgaattaattctgtggaatgtgtgtcagttagggtgtggaaagtccccaggctccccagcaggcagaagtatgcaaagcatgcatctcaattagtcagcaaccaggtgtggaaagtccccaggctccccagcaggcagaagtatgcaaagcatgcatctcaattagtcagcaaccatagtcccgcccctaactccgcccatcccgcccctaactccgcccagttccgcccattctccgccccatggctgactaattttttttatttatgcagaggccgaggccgcctctgcctctgagctattccagaagtagtgaggaggcttttttggaggcctaggcttttgcaaaaagctcccgggagcttgtatatccattttcggatctgatcagcacgtgttgacaattaatcatcggcatagtatatcggcatagtataatacgacaaggtgaggaactaaaccatggccaagttgaccagtgccgttccggtgctcaccgcgcgcgacgtcgccggagcggtcgagttctggaccgaccggctcgggttctcccgggacttcgtggaggacgacttcgccggtgtggtccgggacgacgtgaccctgttcatcagcgcggtccaggaccaggtggtgccggacaacaccctggcctgggtgtgggtgcgcggcctggacgagctgtacgccgagtggtcggaggtcgtgtccacgaacttccgggacgcctccgggccggccatgaccgagatcggcgagcagccgtgggggcgggagttcgccctgcgcgacccggccggcaactgcgtgcacttcgtggccgaggagcaggactgacacgtgctacgagatttcgattccaccgccgccttctatgaaaggttgggcttcggaatcgttttccgggacgccggctggatgatcctccagcgcggggatctcatgctggagttcttcgcccaccccaacttgtttattgcagcttataatggttacaaataaagcaatagcatcacaaatttcacaaataaagcatttttttcactgcattctagttgtggtttgtccaaactcatcaatgtatcttatcatgtctgtataccgtcgacctctagctagagcttggcgtaatcatggtcatagctgtttcctgtgtgaaattgttatccgctcacaattccacacaacatacgagccggaagcataaagtgtaaagcctggggtgcctaatgagtgagctaactcacattaattgcgttgcgctcactgcccgctttccagtcgggaaacctgtcgtgccagctgcattaatgaatcggccaacgcgcggggagaggcggtttgcgtattgggcgctcttccgcttcctcgctcactgactcgctgcgctcggtcgttcggctgcggcgagcggtatcagctcactcaaaggcggtaatacggttatccacagaatcaggggataacgcaggaaagaacatgtgagcaaaaggccagcaaaaggccaggaaccgtaaaaaggccgcgttgctggcgtttttccataggctccgcccccctgacgagcatcacaaaaatcgacgctcaagtcagaggtggcgaaacccgacaggactataaagataccaggcgtttccccctggaagctccctcgtgcgctctcctgttccgaccctgccgcttaccggatacctgtccgcctttctcccttcgggaagcgtggcgctttctcatagctcacgctgtaggtatctcagttcggtgtaggtcgttcgctccaagctgggctgtgtgcacgaaccccccgttcagcccgaccgctgcgccttatccggtaactatcgtcttgagtccaacccggtaagacacgacttatcgccactggcagcagccactggtaacaggattagcagagcgaggtatgtaggcggtgctacagagttcttgaagtggtggcctaactacggctacactagaagaacagtatttggtatctgcgctctgctgaagccagttaccttcggaaaaagagttggtagctcttgatccggcaaacaaaccaccgctggtagcggtggtttttttgtttgcaagcagcagattacgcgcagaaaaaaaggatctcaagaagatcctttgatcttttctacggggtctgacgctcagtggaacgaaaactcacgttaagggattttggtcatgagattatcaaaaaggatcttcacctagatccttttaaattaaaaatgaagttttaaatcaatctaaagtatatatgagtaaacttggtctgacagttaccaatgcttaatcagtgaggcacctatctcagcgatctgtctatttcgttcatccatagttgcctgactccccgtcgtgtagataactacgatacgggagggcttaccatctggccccagtgctgcaatgataccgcgagacccacgctcaccggctccagatttatcagcaataaaccagccagccggaagggccgagcgcagaagtggtcctgcaactttatccgcctccatccagtctattaattgttgccgggaagctagagtaagtagttcgccagttaatagtttgcgcaacgttgttgccattgctacaggcatcgtggtgtcacgctcgtcgtttggtatggcttcattcagctccggttcccaacgatcaaggcgagttacatgatcccccatgttgtgcaaaaaagcggttagctccttcggtcctccgatcgttgtcagaagtaagttggccgcagtgttatcactcatggttatggcagcactgcataattctcttactgtcatgccatccgtaagatgcttttctgtgactggtgagtactcaaccaagtcattctgagaatagtgtatgcggcgaccgagttgctcttgcccggcgtcaatacgggataataccgcgccacatagcagaactttaaaagtgctcatcattggaaaacgttcttcggggcgaaaactctcaaggatcttaccgctgttgagatccagttcgatgtaacccactcgtgcacccaactgatcttcagcatcttttactttcaccagcgtttctgggtgagcaaaaacaggaaggcaaaatgccgcaaaaaagggaataagggcgacacggaaatgttgaatactcatactcttcctttttcaatattattgaagcatttatcagggttattgtctcatgagcggatacatatttgaatgtatttagaaaaataaacaaataggggttccgcgcacatttccccgaaaagtgccacctgacgtcgacggatcgggagatctcccgatcccctatggtgcactctcagtacaatctgctctgatgccgcatagttaagccagtatctgctccctgcttgtgtgttggaggtcgctgagtagtgcgcgagcaaaatttaagctacaacaaggcaaggcttgaccgacaattgcatgaagaatctgcttagggttaggcgttttgcgctgcttcgcgatgtacgggccagatatacgcgttgacattgattattgactagttattaatagtaatcaattacggggtcattagttcatagcccatatatggagttccgcgttacataacttacggtaaatggcccgcctggctgaccgcccaacgacccccgcccattgacgtcaataatgacgtatgttcccatagtaacgccaatagggactttccattgacgtcaatgggtggagtatttacggtaaactgcccacttggcagtacatcaagtgtatcatatgccaagtacgccccctattgacgtcaatgacggtaaatggcccgcctggcattatgcccagtacatgaccttatgggactttcctacttggcagtacatctacgtattagtcatcgctattaccatgg

SEQ ID NO: 86 - DNA, 4104 bp, Artificial Sequence
  Synthetic
atggacaagaagtacagcatcggcctggacatcggcaccaactctgtgggctgggccgtgatcaccgacgagtacaaggtgcccagcaagaaattcaaggtgctgggcaacaccgaccggcacagcatcaagaagaacctgatcggagccctgctgttcgacagcggcgaaacagccgaggccacccggctgaagagaaccgccagaagaagatacaccagacggaagaaccggatctgctatctgcaagagatcttcagcaacgagatggccaaggtggacgacagcttcttccacagactggaagagtccttcctggtggaagaggataagaagcacgagcggcaccccatcttcggcaacatcgtggacgaggtggcctaccacgagaagtaccccaccatctaccacctgagaaagaaactggtggacagcaccgacaaggccgacctgcggctgatctatctggccctggcccacatgatcaagttccggggccacttcctgatcgagggcgacctgaaccccgacaacagcgacgtggacaagctgttcatccagctggtgcagacctacaaccagctgttcgaggaaaaccccatcaacgccagcggcgtggacgccaaggccatcctgtctgccagactgagcaagagcagacggctggaaaatctgatcgcccagctgcccggcgagaagaagaatggcctgttcggaaacctgattgccctgagcctgggcctgacccccaacttcaagagcaacttcgacctggccgaggatgccaaactgcagctgagcaaggacacctacgacgacgacctggacaacctgctggcccagatcggcgaccagtacgccgacctgtttctggccgccaagaacctgtccgacgccatcctgctgagcgacatcctgagagtgaacaccgagatcaccaaggcccccctgagcgcctctatgatcaagagatacgacgagcaccaccaggacctgaccctgctgaaagctctcgtgcggcagcagctgcctgagaagtacaaagagattttcttcgaccagagcaagaacggctacgccggctacattgacggcggagccagccaggaagagttctacaagttcatcaagcccatcctggaaaagatggacggcaccgaggaactgctcgtgaagctgaacagagaggacctgctgcggaagcagcggaccttcgacaacggcagcatcccccaccagatccacctgggagagctgcacgccattctgcggcggcaggaagatttttacccattcctgaaggacaaccgggaaaagatcgagaagatcctgaccttccgcatcccctactacgtgggccctctggccaggggaaacagcagattcgcctggatgaccagaaagagcgaggaaaccatcaccccctggaacttcgaggaagtggtggacaagggcgcttccgcccagagcttcatcgagcggatgaccaacttcgataagaacctgcccaacgagaaggtgctgcccaagcacagcctgctgtacgagtacttcaccgtgtataacgagctgaccaaagtgaaatacgtgaccgagggaatgagaaagcccgccttcctgagcggcgagcagaaaaaggccatcgtggacctgctgttcaagaccaaccggaaagtgaccgtgaagcagctgaaagaggactacttcaagaaaatcgagtgcttcgactccgtggaaatctccggcgtggaagatcggttcaacgcctccctgggcacataccacgatctgctgaaaattatcaaggacaaggacttcctggacaatgaggaaaacgaggacattctggaagatatcgtgctgaccctgacactgtttgaggacagagagatgatcgaggaacggctgaaaacctatgcccacctgttcgacgacaaagtgatgaagcagctgaagcggcggagatacaccggctggggcaggctgagccggaagctgatcaacggcatccgggacaagcagtccggcaagacaatcctggatttcctgaagtccgacggcttcgccaacagaaacttcatgcagctgatccacgacgacagcctgacctttaaagaggacatccagaaagcccaggtgtccggccagggcgatagcctgcacgagcacattgccaatctggccggcagccccgccattaagaagggcatcctgcagacagtgaaggtggtggacgagctcgtgaaagtgatgggccggcacaagcccgagaacatcgtgatcgaaatggccagagagaaccagaccacccagaagggacagaagaacagccgcgagagaatgaagcggatcgaagagggcatcaaagagctgggcagccagatcctgaaagaacaccccgtggaaaacacccagctgcagaacgagaagctgtacctgtactacctgcagaatgggcgggatatgtacgtggaccaggaactggacatcaaccggctgtccgactacgatgtggaccatatcgtgcctcagagctttctgaaggacgactccatcgacaacaaggtgctgaccagaagcgacaagaaccggggcaagagcgacaacgtgccctccgaagaggtcgtgaagaagatgaagaactactggcggcagctgctgaacgccaagctgattacccagagaaagttcgacaatctgaccaaggccgagagaggcggcctgagcgaactggataaggccggcttcatcaagagacagctggtggaaacccggcagatcacaaagcacgtggcacagatcctggactcccggatgaacactaagtacgacgagaatgacaagctgatccgggaagtgaaagtgatcaccctgaagtccaagctggtgtccgatttccggaaggatttccagttttacaaagtgcgcgagatcaacaactaccaccacgcccacgacgcctacctgaacgccgtcgtgggaaccgccctgatcaaaaagtaccctaagctggaaagcgagttcgtgtacggcgactacaaggtgtacgacgtgcggaagatgatcgccaagagcgagcaggaaatcggcaaggctaccgccaagtacttcttctacagcaacatcatgaactttttcaagaccgagattaccctggccaacggcgagatccggaagcggcctctgatcgagacaaacggcgaaaccggggagatcgtgtgggataagggccgggattttgccaccgtgcggaaagtgctgagcatgccccaagtgaatatcgtgaaaaagaccgaggtgcagacaggcggcttcagcaaagagtctatcctgcccaagaggaacagcgataagctgatcgccagaaagaaggactgggaccctaagaagtacggcggcttcgacagccccaccgtggcctattctgtgctggtggtggccaaagtggaaaagggcaagtccaagaaactgaagagtgtgaaagagctgctggggatcaccatcatggaaagaagcagcttcgagaagaatcccatcgactttctggaagccaagggctacaaagaagtgaaaaaggacctgatcatcaagctgcctaagtactccctgttcgagctggaaaacggccggaagagaatgctggcctctgccggcgaactgcagaagggaaacgaactggccctgccctccaaatatgtgaacttcctgtacctggccagccactatgagaagctgaagggctcccccgaggataatgagcagaaacagctgtttgtggaacagcacaagcactacctggacgagatcatcgagcagatcagcgagttctccaagagagtgatcctggccgacgctaatctggacaaagtgctgtccgcctacaacaagcaccgggataagcccatcagagagcaggccgagaatatcatccacctgtttaccctgaccaatctgggagcccctgccgccttcaagtactttgacaccaccatcgaccggaagaggtacaccagcaccaaagaggtgctggacgccaccctgatccaccagagcatcaccggcctgtacgagacacggatcgacctgtctcagctgggaggcgac

SEQ ID NO: 87 - protein, 1368 aa, Artificial Sequence [sequence omitted]

SEQ ID NO: 88 - protein, 31 aa, Homo sapiens
QTAPVPMPDLKNVKSKIGSTENLKHQPGGGK

SEQ ID NO: 89 - protein, 31 aa, Homo sapiens
VQIINKKLDLSNVQSKCGSKDNIKHVPGGGS

SEQ ID NO: 90 - protein, 31 aa, Homo sapiens
VQIVYKPVDLSKVTSKCGSLGNIHHKPGGGQ

SEQ ID NO: 91 - protein, 32 aa, Homo sapiens
VEVKSEKLDFKDRVQSKIGSLDNITHVPGGGN

SEQ ID NO: 92 - DNA, 93 bp, Homo sapiens
cagacagcccccgtgcccatgccagacctgaagaatgtcaagtccaagatcggctccactgagaacctgaagcaccagccgggaggcgggaag

SEQ ID NO: 93 - DNA, 93 bp, Homo sapiens
gtgcagataattaataagaagctggatcttagcaacgtccagtccaagtgtggctcaaaggataatatcaaacacgtcccgggaggcggcagt

SEQ ID NO: 94 - DNA, 93 bp, Homo sapiens
gtgcaaatagtctacaaaccagttgacctgagcaaggtgacctccaagtgtggctcattaggcaacatccatcataaaccaggaggtggccag

SEQ ID NO: 95 - DNA, 96 bp, Homo sapiens
gtggaagtaaaatctgagaagcttgacttcaaggacagagtccagtcgaagattgggtccctggacaatatcacccacgtccctggcggaggaaat

SEQ ID NO: 96 - protein, 133 aa, Homo sapiens
LQTAPVPMPDLKNVKSKIGSTENLKHQPGGGKVQIINKKLDLSNVQSKCGSKDNIKHVPGGGSVQIVYKPVDLSKVTSKCGSLGNIHHKPGGGQVEVKSEKLDFKDRVQSKIGSLDNITHVPGGGNKKIETHK

SEQ ID NO: 97 - DNA, 399 bp, Homo sapiens
ctgcagacagcccccgtgcccatgccagacctgaagaatgtcaagtccaagatcggctccactgagaacctgaagcaccagccgggaggcgggaaggtgcagataattaataagaagctggatcttagcaacgtccagtccaagtgtggctcaaaggataatatcaaacacgtcccgggaggcggcagtgtgcaaatagtctacaaaccagttgacctgagcaaggtgacctccaagtgtggctcattaggcaacatccatcataaaccaggaggtggccaggtggaagtaaaatctgagaagcttgacttcaaggacagagtccagtcgaagattgggtccctggacaatatcacccacgtccctggcggaggaaataaaaagattgaaacccacaag

SEQ ID NO: 98 - protein, 133 aa, Homo sapiens
LQTAPVPMPDLKNVKSKIGSTENLKHQPGGGKVQIINKKLDLSNVQSKCGSKDNIKHVSGGGSVQIVYKPVDLSKVTSKCGSLGNIHHKPGGGQVEVKSEKLDFKDRVQSKIGSLDNITHVPGGGNKKIETHK

SEQ ID NO: 99 - DNA, 399 bp, Homo sapiens
ctgcagacagcccccgtgcccatgccagacctgaagaatgtcaagtccaagatcggctccactgagaacctgaagcaccagccgggaggcgggaaggtgcagataattaataagaagctggatcttagcaacgtccagtccaagtgtggctcaaaggataatatcaaacacgtctcgggaggcggcagtgtgcaaatagtctacaaaccagttgacctgagcaaggtgacctccaagtgtggctcattaggcaacatccatcataaaccaggaggtggccaggtggaagtaaaatctgagaagcttgacttcaaggacagagtccagtcgaagattgggtccctggacaatatcacccacgtccctggcggaggaaataaaaagattgaaacccacaag

SEQ ID NO: 100 - RNA, 72 nt, Artificial Sequence
  Synthetic
aaacagcauagcaaguuaaaauaaggcuaguccguuaucaacuugaaaaaguggcaccgagucggugcuuuu

SEQ ID NO: 101 - RNA, 82 nt, Artificial Sequence; identical to SEQ ID NO: 68
  Synthetic

SEQ ID NO: 102 - RNA, 83 nt, Artificial Sequence
  Synthetic
guuuuagagcuagaaauagcaaguuaaaauaaggcuaguccguuaucaacuugaaaaaguggcaccgagucggugcuuuuuuu

SEQ ID NO: 103 - RNA, 80 nt, Artificial Sequence
  Synthetic
guuuuagagcuagaaauagcaaguuaaaauaaggcuaguccguuaucaacuugaaaaaguggcaccgagucggugcuuuu

SEQ ID NO: 104 - RNA, 92 nt, Artificial Sequence
  Synthetic
guuuaagagcuaugcuggaaacagcauagcaaguuuaaauaaggcuaguccguuaucaacuugaaaaaguggcaccgagucggugcuuuuuu

SEQ ID NO: 105 - DNA, 20 bp, Artificial Sequence
  Synthetic
tgggaggttgtcatcgtgat

SEQ ID NO: 106 - DNA, 20 bp, Artificial Sequence
  Synthetic
cagcctcttgctcaggacgt

SEQ ID NO: 107 - DNA, 20 bp, Artificial Sequence
  Synthetic
cataagccttgtcaaagccc

SEQ ID NO: 108 - DNA, 20 bp, Artificial Sequence
  Synthetic
ggaccacataagccttgtca

SEQ ID NO: 109 - DNA, 20 bp, Artificial Sequence
  Synthetic
catctttctttagcaccaga

SEQ ID NO: 110 - DNA, 20 bp, Artificial Sequence
  Synthetic
ggtcttcatctttctttagc

SEQ ID NO: 111 - DNA, 20 bp, Artificial Sequence
  Synthetic
ccattctcggaagaggtctt

SEQ ID NO: 112 - DNA, 20 bp, Artificial Sequence
  Synthetic
tcagccattctcggaagagg

SEQ ID NO: 113 - DNA, 20 bp, Artificial Sequence
  Synthetic
catgtatccttcagccattc

SEQ ID NO: 114 - DNA, 20 bp, Artificial Sequence
  Synthetic
tgcttggcattggcaccaca

SEQ ID NO: 115 - DNA, 20 bp, Artificial Sequence
  Synthetic
ggactgcttggcattggcac

SEQ ID NO: 116 - DNA, 20 bp, Artificial Sequence
  Synthetic
gaaggcacccaaagcagtcc

SEQ ID NO: 117 - DNA, 20 bp, Artificial Sequence
  Synthetic
tcgaaggcacccaaagcagt

SEQ ID NO: 118 - DNA, 20 bp, Artificial Sequence
  Synthetic
tctcgaaggcacccaaagca

SEQ ID NO: 119 - DNA, 20 bp, Artificial Sequence
  Synthetic
attctcgaaggcacccaaag

SEQ ID NO: 120 - DNA, 20 bp, Artificial Sequence
  Synthetic
caccattctcgaaggcaccc

SEQ ID NO: 121 - DNA, 20 bp, Artificial Sequence
  Synthetic
cacaccattctcgaaggcac

SEQ ID NO: 122 - DNA, 20 bp, Artificial Sequence
  Synthetic
atcacaccattctcgaaggc

SEQ ID NO: 123 - DNA, 20 bp, Artificial Sequence
  Synthetic
agagaacactacaagaaggc

SEQ ID NO: 124 - DNA, 20 bp, Artificial Sequence
  Synthetic
tgcagactctggaaactgtg

SEQ ID NO: 125 - DNA, 20 bp, Artificial Sequence
  Synthetic
ccatagaccctggagtacat

SEQ ID NO: 126 - DNA, 20 bp, Artificial Sequence
  Synthetic
gaaacgatcccagaaagatt

SEQ ID NO: 127 - DNA, 20 bp, Artificial Sequence
  Synthetic
gggactcggctttctgtaat

SEQ ID NO: 128 - DNA, 20 bp, Artificial Sequence
  Synthetic
caacttctcgtccatgatgc

SEQ ID NO: 129 - DNA, 20 bp, Artificial Sequence
  Synthetic
tgctcgatccactggtccag

SEQ ID NO: 130 - DNA, 20 bp, Artificial Sequence
  Synthetic
ctcggagagctgcttgcact

SEQ ID NO: 131 - DNA, 20 bp, Artificial Sequence
  Synthetic
cttgacctgggactcggaga

SEQ ID NO: 132 - DNA, 20 bp, Artificial Sequence
  Synthetic
ccttctcgcagaggctcttg

SEQ ID NO: 133 - DNA, 20 bp, Artificial Sequence
  Synthetic
gtcaggatttctttagcctt

SEQ ID NO: 134 - DNA, 20 bp, Artificial Sequence
  Synthetic
gacatcgaacctcttgaacg

SEQ ID NO: 135 - DNA, 20 bp, Artificial Sequence
  Synthetic
agtgactggacatcgaacct

SEQ ID NO: 136 - DNA, 20 bp, Artificial Sequence
  Synthetic
gtacatctccacacacagtg

SEQ ID NO: 137 - DNA, 20 bp, Artificial Sequence
  Synthetic
caggtaatttgtatctggtg

SEQ ID NO: 138 - DNA, 20 bp, Artificial Sequence
  Synthetic
gtctcccataaacaggtaat

SEQ ID NO: 139 - DNA, 20 bp, Artificial Sequence
  Synthetic
ctctcggtaacgaaccttaa

SEQ ID NO: 140 - DNA, 20 bp, Artificial Sequence
  Synthetic
gtgatgcgctctcggtaacg

SEQ ID NO: 141 - DNA, 20 bp, Artificial Sequence
  Synthetic
attccctcggagtatggtga

SEQ ID NO: 142 - DNA, 20 bp, Artificial Sequence
  Synthetic
ctctcgtgattccctcggag

SEQ ID NO: 143 - DNA, 20 bp, Artificial Sequence
  Synthetic
gaacccataaacctgtgtga

SEQ ID NO: 144 - DNA, 20 bp, Artificial Sequence
  Synthetic
tcgtcgtagaacccataaac

SEQ ID NO: 145 - DNA, 20 bp, Artificial Sequence
  Synthetic
aaggtctgtgaagtatttcc

SEQ ID NO: 146 - DNA, 20 bp, Artificial Sequence
  Synthetic
gtgagaggaagatagtcaaa

SEQ ID NO: 147 - DNA, 20 bp, Artificial Sequence
  Synthetic
ccaaggcagtgagaggaaga

SEQ ID NO: 148 - DNA, 20 bp, Artificial Sequence
  Synthetic
accaccgtgtagacagaaga

SEQ ID NO: 149 - DNA, 20 bp, Artificial Sequence
  Synthetic
cagtgtgtctatggatggtg

SEQ ID NO: 150 - DNA, 20 bp, Artificial Sequence
  Synthetic
tcgagtgctcggatgtgatc

SEQ ID NO: 151 - DNA, 20 bp, Artificial Sequence
  Synthetic
gtcacacattggaccctcat

SEQ ID NO: 152 - DNA, 20 bp, Artificial Sequence
  Synthetic
ccaccacggtcatctggatc

SEQ ID NO: 153 - DNA, 20 bp, Artificial Sequence
  Synthetic
gccaaaggtataaccagctc

SEQ ID NO: 154 - DNA, 20 bp, Artificial Sequence
  Synthetic
tgaggccattggcatgatta

SEQ ID NO: 155 - DNA, 20 bp, Artificial Sequence
  Synthetic
tggacaccaacgtgaggcca

SEQ ID NO: 156 - DNA, 20 bp, Artificial Sequence
  Synthetic
gttatatccctccatcacca

SEQ ID NO: 157 - DNA, 20 bp, Artificial Sequence
  Synthetic
tggcaccagttatatccctc

SEQ ID NO: 158 - DNA, 20 bp, Artificial Sequence
  Synthetic
acgttccggtcatggcacca

SEQ ID NO: 159 - DNA, 20 bp, Artificial Sequence
  Synthetic
ttgttactacgttccggtca

SEQ ID NO: 160 - DNA, 20 bp, Artificial Sequence
  Synthetic
agcaatagtttggagcactg

SEQ ID NO: 161 - DNA, 20 bp, Artificial Sequence
  Synthetic
taccacaacgatagcaatag

SEQ ID NO: 162 - DNA, 20 bp, Artificial Sequence
  Synthetic
agcttggttaccacaacgat

SEQ ID NO: 163 - DNA, 20 bp, Artificial Sequence
  Synthetic
agtgtcgtcaagttccatga

SEQ ID NO: 164 - DNA, 20 bp, Artificial Sequence
  Synthetic
gctgggtcaaactgcaagaa

SEQ ID NO: 165 - DNA, 20 bp, Artificial Sequence
  Synthetic
acggttcatggcaatactgt

SEQ ID NO: 166 - DNA, 20 bp, Artificial Sequence
  Synthetic
gtcaatatacggttcatggc

SEQ ID NO: 167 - DNA, 20 bp, Artificial Sequence
  Synthetic
tgttgctcttcccatttcca

SEQ ID NO: 168 - DNA, 20 bp, Artificial Sequence
  Synthetic
tttggtccgtgtgaaaacaa

SEQ ID NO: 169 - DNA, 20 bp, Artificial Sequence
  Synthetic
caagagtttcagtcgagcca

SEQ ID NO: 170 - DNA, 20 bp, Artificial Sequence
  Synthetic
gtcatctggattcaagagtt

SEQ ID NO: 171 - DNA, 20 bp, Artificial Sequence
  Synthetic
agtccttgaggtgccctgga

SEQ ID NO: 172 - DNA, 20 bp, Artificial Sequence
  Synthetic
ggcctgctgagtttgtttcc

SEQ ID NO: 173 - DNA, 20 bp, Artificial Sequence
  Synthetic
agggttcaagcccacactgt

SEQ ID NO: 174 - DNA, 20 bp, Artificial Sequence
  Synthetic
tgggtggacactggatgcta

SEQ ID NO: 175 - DNA, 20 bp, Artificial Sequence
  Synthetic
gtggttgtcattcctggtag

SEQ ID NO: 176 - DNA, 20 bp, Artificial Sequence
  Synthetic
agggccatcctcatatactg

SEQ ID NO: 177 - DNA, 20 bp, Artificial Sequence
  Synthetic
ctcatgtctcacagggccat

SEQ ID NO: 178 - DNA, 20 bp, Artificial Sequence
  Synthetic
taagggcgtagttttgttgg

SEQ ID NO: 179 - DNA, 20 bp, Artificial Sequence
  Synthetic
ttcagccaggcacaagccat

SEQ ID NO: 180 - DNA, 20 bp, Artificial Sequence
  Synthetic
gtaactgtttgctcgttctt

SEQ ID NO: 181 - DNA, 20 bp, Artificial Sequence
  Synthetic
ggaagcctggttctctttgg

SEQ ID NO: 182 - DNA, 20 bp, Artificial Sequence
  Synthetic
acgcataaactcagggttct

SEQ ID NO: 183 - DNA, 20 bp, Artificial Sequence
  Synthetic
catgttgtcatctgggtaca

SEQ ID NO: 184 - DNA, 20 bp, Artificial Sequence
  Synthetic
gtcaacaacgtagaggatgc

SEQ ID NO: 185 - DNA, 20 bp, Artificial Sequence
  Synthetic
caggagtggcacatagtagt

SEQ ID NO: 186 - DNA, 20 bp, Artificial Sequence
  Synthetic
agtatttgaggcttcagctt

SEQ ID NO: 187 - DNA, 20 bp, Artificial Sequence
  Synthetic
aggtcccacgaaagctctca

SEQ ID NO: 188 - DNA, 20 bp, Artificial Sequence
  Synthetic
atcttctgctttggatggac

SEQ ID NO: 189 - DNA, 20 bp, Artificial Sequence
  Synthetic
tttctttcgaggtggagttt

SEQ ID NO: 190 - DNA, 20 bp, Artificial Sequence
  Synthetic
aatgcctcgttctgggtcag

SEQ ID NO: 191 - DNA, 20 bp, Artificial Sequence
  Synthetic
tccaactctctcaatgcctc

SEQ ID NO: 192 - DNA, 20 bp, Artificial Sequence
  Synthetic
ttcccagtattcaacccagg

SEQ ID NO: 193 - DNA, 20 bp, Artificial Sequence
  Synthetic
acatcccagaaattcccagt

SEQ ID NO: 194 - DNA, 20 bp, Artificial Sequence
  Synthetic
gcagccttcattttctcgta

SEQ ID NO: 195 - DNA, 20 bp, Artificial Sequence
  Synthetic
ctttccactgccaaaatctg

SEQ ID NO: 196 - DNA, 20 bp, Artificial Sequence
  Synthetic
cacggagatggagttgctgt

SEQ ID NO: 197 - DNA, 20 bp, Artificial Sequence
  Synthetic
gggctgactctgacttggaa

SEQ ID NO: 198 - DNA, 20 bp, Artificial Sequence
  Synthetic
agaggtttggaacttatcag

SEQ ID NO: 199 - DNA, 20 bp, Artificial Sequence
  Synthetic
agttccaactgaggtttctc

SEQ ID NO: 200 - DNA, 20 bp, Artificial Sequence
  Synthetic
gtcactgtctgctgcaccct

SEQ ID NO: 201 - DNA, 20 bp, Artificial Sequence
  Synthetic
agatgccagcaagtcactgt

SEQ ID NO: 202 - DNA, 20 bp, Artificial Sequence
  Synthetic
agtgttggtcctgacttgct

SEQ ID NO: 203 - DNA, 20 bp, Artificial Sequence
  Synthetic
gagtataggttccagaccag

SEQ ID NO: 204 - DNA, 20 bp, Artificial Sequence
  Synthetic
ggtggaatctaccgtggcag

SEQ ID NO: 205 - DNA, 20 bp, Artificial Sequence
  Synthetic
ttttgatggttcctctccag

SEQ ID NO: 206 - DNA, 20 bp, Artificial Sequence
  Synthetic
cgcacactcaagagctgcta

SEQ ID NO: 207 - DNA, 20 bp, Artificial Sequence
  Synthetic
tgggtacagaccagggtcaa

SEQ ID NO: 208 - DNA, 20 bp, Artificial Sequence
  Synthetic
gtctgagggcgagtagcaca

SEQ ID NO: 209 - DNA, 20 bp, Artificial Sequence
  Synthetic
cttccctttgagtgcaggac

SEQ ID NO: 210 - DNA, 20 bp, Artificial Sequence
  Synthetic
atgagagcaatcgagatcca

SEQ ID NO: 211 - DNA, 20 bp, Artificial Sequence
  Synthetic
gccagaagaggaggaggtgt

SEQ ID NO: 212 - DNA, 20 bp, Artificial Sequence
  Synthetic
cccatgtgctggactgtagc

SEQ ID NO: 213 - DNA, 20 bp, Artificial Sequence
  Synthetic
atgaatcccaggagtaagct

SEQ ID NO: 214 - DNA, 20 bp, Artificial Sequence
  Synthetic
ctcacttgtctatgcctttg

SEQ ID NO: 215 - RNA, 20 nt, Artificial Sequence
  Synthetic
ugggagguugucaucgugau

SEQ ID NO: 216 - RNA, 20 nt, Artificial Sequence
  Synthetic
cagccucuugcucaggacgu

SEQ ID NO: 217 - RNA, 20 nt, Artificial Sequence
  Synthetic
cauaagccuugucaaagccc

SEQ ID NO: 218 - RNA, 20 nt, Artificial Sequence
  Synthetic
ggaccacauaagccuuguca

SEQ ID NO: 219 - RNA, 20 nt, Artificial Sequence
  Synthetic
caucuuucuuuagcaccaga

SEQ ID NO: 220 - RNA, 20 nt, Artificial Sequence
  Synthetic
ggucuucaucuuucuuuagc

SEQ ID NO: 221 - RNA, 20 nt, Artificial Sequence
  Synthetic
ccauucucggaagaggucuu

SEQ ID NO: 222 - RNA, 20 nt, Artificial Sequence
  Synthetic
ucagccauucucggaagagg

SEQ ID NO: 223 - RNA, 20 nt, Artificial Sequence
  Synthetic
cauguauccuucagccauuc

SEQ ID NO: 224 - RNA, 20 nt, Artificial Sequence
  Synthetic
ugcuuggcauuggcaccaca

SEQ ID NO: 225 - RNA, 20 nt, Artificial Sequence
  Synthetic
ggacugcuuggcauuggcac

SEQ ID NO: 226 - RNA, 20 nt, Artificial Sequence
  Synthetic
gaaggcacccaaagcagucc

SEQ ID NO: 227 - RNA, 20 nt, Artificial Sequence
  Synthetic
ucgaaggcacccaaagcagu

SEQ ID NO: 228 - RNA, 20 nt, Artificial Sequence
  Synthetic
ucucgaaggcacccaaagca

SEQ ID NO: 229 - RNA, 20 nt, Artificial Sequence
  Synthetic
auucucgaaggcacccaaag

SEQ ID NO: 230 - RNA, 20 nt, Artificial Sequence
  Synthetic
caccauucucgaaggcaccc

SEQ ID NO: 231 - RNA, 20 nt, Artificial Sequence
  Synthetic
cacaccauucucgaaggcac

SEQ ID NO: 232 - RNA, 20 nt, Artificial Sequence
  Synthetic
aucacaccauucucgaaggc

SEQ ID NO: 233 - RNA, 20 nt, Artificial Sequence
  Synthetic
agagaacacuacaagaaggc

SEQ ID NO: 234 - RNA, 20 nt, Artificial Sequence
  Synthetic
ugcagacucuggaaacugug

SEQ ID NO: 235 - RNA, 20 nt, Artificial Sequence
  Synthetic
ccauagacccuggaguacau

SEQ ID NO: 236 - RNA, 20 nt, Artificial Sequence
  Synthetic
gaaacgaucccagaaagauu

SEQ ID NO: 237 - RNA, 20 nt, Artificial Sequence
  Synthetic
gggacucggcuuucuguaau

SEQ ID NO: 238 - RNA, 20 nt, Artificial Sequence
  Synthetic
caacuucucguccaugaugc

SEQ ID NO: 239 - RNA, 20 nt, Artificial Sequence
  Synthetic
ugcucgauccacugguccag

SEQ ID NO: 240 - RNA, 20 nt, Artificial Sequence
  Synthetic
cucggagagcugcuugcacu

SEQ ID NO: 241 - RNA, 20 nt, Artificial Sequence
  Synthetic
cuugaccugggacucggaga

SEQ ID NO: 242 - RNA, 20 nt, Artificial Sequence
  Synthetic
ccuucucgcagaggcucuug

SEQ ID NO: 243 - RNA, 20 nt, Artificial Sequence
  Synthetic
gucaggauuucuuuagccuu

SEQ ID NO: 244 - RNA, 20 nt, Artificial Sequence
  Synthetic
gacaucgaaccucuugaacg

SEQ ID NO: 245 - RNA, 20 nt, Artificial Sequence
  Synthetic
agugacuggacaucgaaccu

SEQ ID NO: 246 - RNA, 20 nt, Artificial Sequence
  Synthetic
guacaucuccacacacagug

SEQ ID NO: 247 - RNA, 20 nt, Artificial Sequence
  Synthetic
cagguaauuuguaucuggug

SEQ ID NO: 248 - RNA, 20 nt, Artificial Sequence
  Synthetic
gucucccauaaacagguaau

SEQ ID NO: 249 - RNA, 20 nt, Artificial Sequence
  Synthetic
cucucgguaacgaaccuuaa

SEQ ID NO: 250 - RNA, 20 nt, Artificial Sequence
  Synthetic
gugaugcgcucucgguaacg

SEQ ID NO: 251 - RNA, 20 nt, Artificial Sequence
  Synthetic
auucccucggaguaugguga

SEQ ID NO: 252 - RNA, 20 nt, Artificial Sequence
  Synthetic
cucucgugauucccucggag

SEQ ID NO: 253 - RNA, 20 nt, Artificial Sequence
  Synthetic
gaacccauaaaccuguguga

SEQ ID NO: 254 - RNA, 20 nt, Artificial Sequence
  Synthetic
ucgucguagaacccauaaac

SEQ ID NO: 255 - RNA, 20 nt, Artificial Sequence
  Synthetic
aaggucugugaaguauuucc

SEQ ID NO: 256 - RNA, 20 nt, Artificial Sequence
  Synthetic
gugagaggaagauagucaaa

SEQ ID NO: 257 - RNA, 20 nt, Artificial Sequence
  Synthetic
ccaaggcagugagaggaaga

SEQ ID NO: 258 - RNA, 20 nt, Artificial Sequence
  Synthetic
accaccguguagacagaaga

SEQ ID NO: 259 - RNA, 20 nt, Artificial Sequence
  Synthetic
cagugugucuauggauggug

SEQ ID NO: 260 - RNA, 20 nt, Artificial Sequence
  Synthetic
ucgagugcucggaugugauc

SEQ ID NO: 261 - RNA, 20 nt, Artificial Sequence
  Synthetic
gucacacauuggacccucau

SEQ ID NO: 262 - RNA, 20 nt, Artificial Sequence
  Synthetic
ccaccacggucaucuggauc

SEQ ID NO: 263 - RNA, 20 nt, Artificial Sequence
  Synthetic
gccaaagguauaaccagcuc

SEQ ID NO: 264 - RNA, 20 nt, Artificial Sequence
  Synthetic
ugaggccauuggcaugauua

SEQ ID NO: 265 - RNA, 20 nt, Artificial Sequence
  Synthetic
uggacaccaacgugaggcca

SEQ ID NO: 266 - RNA, 20 nt, Artificial Sequence
  Synthetic
guuauaucccuccaucacca

SEQ ID NO: 267 - RNA, 20 nt, Artificial Sequence
  Synthetic
uggcaccaguuauaucccuc

SEQ ID NO: 268 - RNA, 20 nt, Artificial Sequence
  Synthetic
acguuccggucauggcacca

SEQ ID NO: 269 - RNA, 20 nt, Artificial Sequence
  Synthetic
uuguuacuacguuccgguca

SEQ ID NO: 270 - RNA, 20 nt, Artificial Sequence
  Synthetic
agcaauaguuuggagcacug

SEQ ID NO: 271 - RNA, 20 nt, Artificial Sequence
  Synthetic
uaccacaacgauagcaauag

SEQ ID NO: 272 - RNA, 20 nt, Artificial Sequence
  Synthetic
agcuugguuaccacaacgau

SEQ ID NO: 273 - RNA, 20 nt, Artificial Sequence
  Synthetic
agugucgucaaguuccauga

SEQ ID NO: 274 - RNA, 20 nt, Artificial Sequence
  Synthetic
gcugggucaaacugcaagaa

SEQ ID NO: 275 - RNA, 20 nt, Artificial Sequence
  Synthetic
acgguucauggcaauacugu

SEQ ID NO: 276 - RNA, 20 nt, Artificial Sequence
  Synthetic
gucaauauacgguucauggc

SEQ ID NO: 277 - RNA, 20 nt, Artificial Sequence
  Synthetic
uguugcucuucccauuucca

SEQ ID NO: 278 - RNA, 20 nt, Artificial Sequence
  Synthetic
uuugguccgugugaaaacaa

SEQ ID NO: 279 - RNA, 20 nt, Artificial Sequence
  Synthetic
caagaguuucagucgagcca

SEQ ID NO: 280 - RNA, 20 nt, Artificial Sequence
  Synthetic
gucaucuggauucaagaguu

SEQ ID NO: 281 - RNA, 20 nt, Artificial Sequence
  Synthetic
aguccuugaggugcccugga

SEQ ID NO: 282 - RNA, 20 nt, Artificial Sequence
  Synthetic
ggccugcugaguuuguuucc

SEQ ID NO: 283 - RNA, 20 nt, Artificial Sequence
  Synthetic
aggguucaagcccacacugu

SEQ ID NO: 284 - RNA, 20 nt, Artificial Sequence
  Synthetic
uggguggacacuggaugcua

SEQ ID NO: 285 - RNA, 20 nt, Artificial Sequence
  Synthetic
gugguugucauuccugguag

SEQ ID NO: 286 - RNA, 20 nt, Artificial Sequence
  Synthetic
agggccauccucauauacug

SEQ ID NO: 287 - RNA, 20 nt, Artificial Sequence
  Synthetic
cucaugucucacagggccau

SEQ ID NO: 288 - RNA, 20 nt, Artificial Sequence
  Synthetic
uaagggcguaguuuuguugg

SEQ ID NO: 289 - RNA, 20 nt, Artificial Sequence
  Synthetic
uucagccaggcacaagccau

SEQ ID NO: 290 - RNA, 20 nt, Artificial Sequence
  Synthetic
guaacuguuugcucguucuu

SEQ ID NO: 291 - RNA, 20 nt, Artificial Sequence
  Synthetic
ggaagccugguucucuuugg

SEQ ID NO: 292 - RNA, 20 nt, Artificial Sequence
  Synthetic
acgcauaaacucaggguucu

SEQ ID NO: 293 - RNA, 20 nt, Artificial Sequence
  Synthetic
cauguugucaucuggguaca

SEQ ID NO: 294 - RNA, 20 nt, Artificial Sequence
  Synthetic
gucaacaacguagaggaugc

SEQ ID NO: 295 - RNA, 20 nt, Artificial Sequence
  Synthetic
caggaguggcacauaguagu

SEQ ID NO: 296 - RNA, 20 nt, Artificial Sequence
  Synthetic
aguauuugaggcuucagcuu

SEQ ID NO: 297 - RNA, 20 nt, Artificial Sequence
  Synthetic
aggucccacgaaagcucuca

SEQ ID NO: 298 - RNA, 20 nt, Artificial Sequence
  Synthetic
aucuucugcuuuggauggac

SEQ ID NO: 299 - RNA, 20 nt, Artificial Sequence
  Synthetic
uuucuuucgagguggaguuu

SEQ ID NO: 300 - RNA, 20 nt, Artificial Sequence
  Synthetic
aaugccucguucugggucag

SEQ ID NO: 301 - RNA, 20 nt, Artificial Sequence
  Synthetic
uccaacucucucaaugccuc

SEQ ID NO: 302 - RNA, 20 nt, Artificial Sequence
  Synthetic
uucccaguauucaacccagg

SEQ ID NO: 303 - RNA, 20 nt, Artificial Sequence
  Synthetic
acaucccagaaauucccagu

SEQ ID NO: 304 - RNA, 20 nt, Artificial Sequence
  Synthetic
gcagccuucauuuucucgua

SEQ ID NO: 305 - RNA, 20 nt, Artificial Sequence
  Synthetic
cuuuccacugccaaaaucug

SEQ ID NO: 306 - RNA, 20 nt, Artificial Sequence
  Synthetic
cacggagauggaguugcugu

SEQ ID NO: 307 - RNA, 20 nt, Artificial Sequence
  Synthetic
gggcugacucugacuuggaa

SEQ ID NO: 308 - RNA, 20 nt, Artificial Sequence
  Synthetic
agagguuuggaacuuaucag

SEQ ID NO: 309 - RNA, 20 nt, Artificial Sequence
  Synthetic
aguuccaacugagguuucuc

SEQ ID NO: 310 - RNA, 20 nt, Artificial Sequence
  Synthetic
gucacugucugcugcacccu

SEQ ID NO: 311 - RNA, 20 nt, Artificial Sequence
  Synthetic
agaugccagcaagucacugu

SEQ ID NO: 312 - RNA, 20 nt, Artificial Sequence
  Synthetic
aguguugguccugacuugcu

SEQ ID NO: 313 - RNA, 20 nt, Artificial Sequence
  Synthetic
gaguauagguuccagaccag

SEQ ID NO: 314 - RNA, 20 nt, Artificial Sequence
  Synthetic
gguggaaucuaccguggcag

SEQ ID NO: 315 - RNA, 20 nt, Artificial Sequence
  Synthetic
uuuugaugguuccucuccag

SEQ ID NO: 316 - RNA, 20 nt, Artificial Sequence
  Synthetic
cgcacacucaagagcugcua

SEQ ID NO: 317 - RNA, 20 nt, Artificial Sequence
  Synthetic
uggguacagaccagggucaa

SEQ ID NO: 318 - RNA, 20 nt, Artificial Sequence
  Synthetic
gucugagggcgaguagcaca

SEQ ID NO: 319 - RNA, 20 nt, Artificial Sequence
  Synthetic
cuucccuuugagugcaggac

SEQ ID NO: 320 - RNA, 20 nt, Artificial Sequence
  Synthetic
augagagcaaucgagaucca

SEQ ID NO: 321 - RNA, 20 nt, Artificial Sequence
  Synthetic
gccagaagaggaggaggugu

SEQ ID NO: 322 - RNA, 20 nt, Artificial Sequence
  Synthetic
cccaugugcuggacuguagc

SEQ ID NO: 323 - RNA, 20 nt, Artificial Sequence
  Synthetic
augaaucccaggaguaagcu

SEQ ID NO: 324 - RNA, 20 nt, Artificial Sequence
  Synthetic
cucacuugucuaugccuuug